European Patent Specification EP 2 941 488 B1, published March 22, 2023. Title: METHODS OF INTRODUCING dsRNA TO PLANT SEEDS FOR MODULATING GENE EXPRESSION. Applicant: A.B. Seeds Ltd. Avniel, Amir Lidor-Nili, Efrat Maor, Rudy Meir, Ofir Noivirt-Brik, Orly. The sequence listing filed with the application follows.

SEQUENCE LISTING (220 sequences)

SEQ ID NO: 1 - DNA, 20 bp, Artificial Sequence
  polynucleotide sequence or in vitro generated dsRNA
taatacgactcactataggg

SEQ ID NO: 2 - DNA, 19 bp, artificial Sequence
  polynucleotide sequence or in vitro generated dsRNA
ggtgctctgaacgtggatg

SEQ ID NO: 3 - DNA, 22 bp, artificial Sequence
  polynucleotide sequence or in vitro generated dsRNA
catcatcgccatcctcattctc

SEQ ID NO: 4 - DNA, 40 bp, artificial Sequence
  polynucleotide sequence or in vitro generated dsRNA
taatacgactcactataggggaagaccctcgaaactaagc

SEQ ID NO: 5 - DNA, 40 bp, artificial Sequence
  polynucleotide sequence or in vitro generated dsRNA
taatacgactcactatagggggtaagcggcattctaaacc

SEQ ID NO: 6 - DNA, 20 bp, artificial Sequence
  polynucleotide sequence or in vitro generated dsRNA
actcagcagtcgtaggattg

SEQ ID NO: 7 - DNA, 20 bp, artificial Sequence
  polynucleotide sequence or in vitro generated dsRNA
cttcttatgttcccgtcagg

SEQ ID NO: 8 - RNA, 616 nt, CGMMV
uaauacgacucacuauaggggguaagcggcauucuaaaccuccaaaucggagguuggacucugcuucugaagaguccaguucuguuucuuuugaagauggcuuacaauccgaucacaccuagcaaacuuauugcguuuagugcuucuuauguucccgucaggacuuuacuuaauuuucuaguugcuucacaagguaccgcuuuccagacucaagcgggaagagauucuuuccgcgagucccugucugcguuacccucgucugucguagauauuaauucuagauucccagaugcggguuuuuacgcuuuccucaacgguccuguguugaggccuaucuucguuucgcuucucagcuccacggauacgcguaauagggucauugagguuguagauccuagcaauccuacgacugcugagucgcuuaacgccguaaagcguacugaugacgcgucuacggccgcuagggcugagauagauaauuuaauagagucuauuucuaaggguuuugauguuuacgauagggcuucauuugaagccgcguuuucgguagucuggucagaggcuaccaccucgaaagcuuaguuucgagggucuuccccuauagugagucguauua

SEQ ID NO: 9 - DNA, 40 bp, artificial Sequence
  polynucleotide sequence or in vitro generated dsRNA
taatacgactcactatagggcatcaccatcgaccctaaac

SEQ ID NO: 10 - DNA, 40 bp, artificial Sequence
  polynucleotide sequence or in vitro generated dsRNA
taatacgactcactataggggctttaccgccactaagaac

SEQ ID NO: 11 - RNA, 598 nt, CGMMV
uaauacgacucacuauaggggcuuuaccgccacuaagaacucuguacacucccuugcggguggucugaggcuucuugaauuggaauauaugaugaugcaagugcccuacggcucaccuuguuaugacaucggcgguaacuauacgcagcacuuguucaaagguagaucauaugugcauugcugcaauccgugccuagaucuuaaagauguugcgaggaaugugauguacaacgauaugaucacgcaacauguacagaggcacaagggaucuggcgggugcagaccucuuccaacuuuccagauagaugcauucaggagguacgauaguucucccugugcggucaccuguucagacguuuuccaagaguguuccuaugauuuugggagugguagggauaaucaugcagucucguugcauucaaucuacgauaucccuuauucuucgaucggaccugcucuucauaggaaaaaugugcgaguuuguuaugcagccuuucauuucucggaggcauugcuuuuagguucgccuguagguaauuuaaauaguauuggggcucaguuuagggucgauggugaugcccuauagugagucguauua

SEQ ID NO: 12 - DNA, 19 bp, artificial Sequence
  polynucleotide sequence or in vitro generated dsRNA
ggtgctctgaacgtggatg

SEQ ID NO: 13 - DNA, 22 bp, artificial Sequence
  polynucleotide sequence or in vitro generated dsRNA
catcatcgccatcctcattctc

SEQ ID NO: 14 - DNA, 43 bp, artificial Sequence
  polynucleotide sequence or in vitro generated dsRNA
taatacgactcactatagggagcattcccggcgggatagtctg

SEQ ID NO: 15 - DNA, 43 bp, artificial Sequence; identical to SEQ ID NO: 14
  polynucleotide sequence or in vitro generated dsRNA

SEQ ID NO: 16 - DNA, 20 bp, artificial Sequence
  polynucleotide sequence or in vitro generated dsRNA
cagcgcgaagtctttatacc

SEQ ID NO: 17 - DNA, 20 bp, artificial Sequence
  polynucleotide sequence or in vitro generated dsRNA
ctttgccgtaatgagtgacc

SEQ ID NO: 18 - DNA, 20 bp, artificial Sequence
  polynucleotide sequence or in vitro generated dsRNA
ccataaccctggaggttgag

SEQ ID NO: 19 - DNA, 20 bp, artificial Sequence
  polynucleotide sequence or in vitro generated dsRNA
atcagacgctgctggtctgg

SEQ ID NO: 20 - RNA, 443 nt, Escherichia coli
uaauacgacucacuauagggagaucgacggccugugggcauucagucuggaucgcgaaaacuguggaauugaucagcguuggugggaaagcgcguuacaagaaagccgggcuauugcugugccaggcaguuuuaacgaucaguucgccgaugcagauauucguaauuaugcgggcaacgucugguaucagcgcgaagucuuuauaccgaaagguugggcaggccagcguaucgugcugcguuucgaugcggucacucauuacggcaaagugugggucaauaaucaggaagugauggagcaucagggcggcuauacgccauuugaagccgaugucacgccguauguuauugccgggaaaaguguacguaucaccguuugugugaacaacgaacugaacuggcagacuaucccgccgggaaugcucccuauagugagucguauua

SEQ ID NO: 21 - DNA, 2070 bp, Spodoptera littoralis
atgtcagacagcgcacaggacgttctacaggatgcggtagccggcgccgccgctgctgctgccgatgccgctgatggatcgctgtttagcacctttgatataattgttctcgttatcttattgggaggcaccatctggtggctatacaactccaaaaaggaaaacaaaaaagatgaaattctgctgagcaaatattccatccaggctgcgggatccattcaagttactgaaaattcttttataaacaaactaaagtcatctggaagaagtttagttgtattctatgggtctcaaacgggtactggtgaggagttcgcgggacgtcttgccaaggagggcatacgatacaagatgaagggtatggttgctgatcccgaagaatgtgatgtggaagaacttatgaaactccaagaaataccgaattcattagctgtgttctgtatggcaacatatggtgaaggagatcccacagacaactctatggagttttatgaatggataaagaacggagaaccggacctaactggtttaaattatgccgtgtttggccttggcaacaagacatatgaacattacaatgcggttgctatatatctagataaacgtcttgaagaacttggcgctacaagagtctttgaacttgggcttggagatgatgacgctaatattgaagatgactttatcacctggaaagaaaagttctggccagctgtatgtgagaaattcaatattgagagcactggtgaagaagagttgattcgtcagttccgtcttgttactcacggacctgatgacatacaacctaacaacatatttactggagaaattgccagattacactccttacaagtccagaggccaccttatgatgccaagaatccattccttgctcaaatcacagttaatagagaattacataagggtggagataggtcttgtatccatgtcgaattggatatttcagactccaaaatgcgatatgaagcaggtgatcatgtggctgtgtacccaataaatgactctaaccttgtagatcgtctaggacaattaacaggggccaaccttgacgagatcttctctctcatcaacactgaccaggaaagcagcaaaaagcatcctttcccttgcccaacctcctatcgcactgcattatcacactatgttgagattactgcattgccccgtactcacatattaagagagttggttgaatactgtacagatgaagaagacaaaaagaaattgatgctcatggcaactaattctcaagagggcaaggccatgtaccaatcatttattgtagaggcttgcagaaatattgtgcacatcttggaagatgtaccatcttgtaaacctccactggaccacttgtgtgaacttttacctcgcctacaaccaagatactactccatctcatccagtcctaagatgtatccagagacagtgcatattactgcagtcgttgttcaatataaaacacctacgggtcgcgtcaacaaaggtgttacgacaacatggttagcagataacaaacccgaacccggcaagcctcttcctcgtgtacccgtatttatcagaaaatcacaattccgattacccctgcaaagtcaaacccccataataatggtcggtcctggtacaggattagctcctttccgtggattcttgcaagagcgtgctttcgcgcgtgcgaatggcaaagaagtgggagacaatgttctatactttggatgcagacatcgcgaccaggattacatttatcaagaggaacttgagaaatacgagcaaaatggtgatgtcaaattgaacctagcattctctcgtgatcaaaaagaaaaagtgtatgtaacacatttactagaaaaagatatggatctcttatgggatgtcatcggtaatcgtaatggacatttctacatttgcggggacgctaagaatatggctgttgacgtaaggaatattgtcttaaagactatccaactaaaaggtggacgcacagaagctgaagctgcacaatttatcaagaagcttgagtctatgaagaaatattctgctgacgtatggagttaa

SEQ ID NO: 22 - DNA, 817 bp, Spodoptera littoralis
acatctggtatcgacgccaagaacactctctgtgagtttaccggcgatatcctgcgtactcccgtctctgaagatatgttgggtcgtgtattcaacggctccggaaagcccattgacaagggtcccccaatcctcgccgaggacttcttggacatccagggacagcccatcaacccatggtcccgtatctaccccgaggagatgatccagactggtatctccgctatcgacgtgatgaactccattgctcgtggtcagaagatccccatcttctctgccgctggtctgccccacaatgaaattgccgcccagatctgtagacaggccggtcttgttaagatccccggcaaatcagtgttggatgaccacgaggacaacttcgccatcgtattcgcagctatgggtgtgaacatggaaaccgcccggttcttcaaacaggacttcgaagagaacggttctatggagaacgtgtgcctgttcttgaacttggccaatgaccccactattgagagaattatcacaccccgtcttgctttgactgctgccgagttcttggcctaccagtgcgagaaacacgtgttggtcatcttgactgacatgtcctcatacgccgaggctctgcgtgaggtgtccgccgcccgtgaggaggtacccggacgtcgtggtttcccaggttacatgtacaccgatttggccaccatctacgagcgtgccggacgtgtagagggcaggaatggatccatcacccagatccccattctgactatgcccaacgacgacatcacccatcctattcctgatttgacgggatatatta

SEQ ID NO: 23 - DNA, 1532 bp, Spodoptera littoralis
cattgaagcgacagctgcactgctcgctagttctcaagtaatcattatcaggtgaaagaaacgaaaatgttggcttatatataagttgtgaacagtgaacctttacaatatattaatatcattcaagacatggaaaaaaacaataaatcaaagcaaaatgtggaaaatataaatactccaactgcttcggggtcagctgctacttcagtggcatccaatggccccgcctcaacattaacgctattcaagagcggaccgcgtgaggctaaaattcgacccctcgcgccattaatgctcccgacgcaaagttacgactcaaacgccggctctccggcttcgtcaccatccacccctcgttcttcatcttctttctccatcgataaaaccgacaatcacgacacctttggcttcagtgcggacacggctgatatgagaaaagaggatgaacgtatgaaaacatttgaaaaatggcccgtcagtttcctaaccggacagcaacttgctcgaaatggattttactacctaggccgtggagatgaagcccgttgcgccttctgtaaagtggagattatgaggtgggttgagggcgatgaccctgcgaaggaccatcagcgttgggcgccacagtgcccattcgtgcgcaagctcaacggtagtgccagcagcgacacgggtagttcgggccaggacgaatgtggggcccgcgccactccctccggtacctctccgccacgtatggccggtcccgtgcacccacgatatgcgtctgaagccgcacgactacgtagctttaaagactggccacgatgcatgcggcaaaaacctgaagaactcgcagaggctggctttttttacactggtcagggagacaaaaccaagtgtttttactgcgatggtggattaaaagattgggagaaccatgacgtaccctgggaacaacatgcacggtggtttgaccgttgcgcctacgtgcaattggtgaagggtcgagaatacgttcaaaaggtgatttctgaggcttgtgaggtatccgcatcggaagcagaacgtgatgttgctccctcacgaactaccagcgagtccagcgcgccagttgagacgccggagaactcagtcgacgactcaaagttgtgtaaaatctgttacgcggaagagcgtaacgtgtgcttcgtgccgtgcggccacgtggtggcttgcgccaagtgcgcgctggcagccgacaagtgccccatgtgccgcaggacgtttcagaatgcagtgcgattatatttctcgtgagaagagccgccaatttgaaggctcgattctagtcttaagggacggccggatagagctgtgtgctgaaaccacgagctcggaagccacgtttccacaggcggagtaacctattaaaacatattgtttgatagtttcgataggaactcgctcgctagtgtagcaaaagacgaaattgagagtcctcaggagtaagacagatatatttaggtatagtgaattataaaatacttagttagcaaaaaaaaaaaaaaaaa

SEQ ID NO: 24 - DNA, 5207 bp, Spodoptera exigua
gagtgagcgcgcggcctaccgaccgaacgcacgcgcaaaccatgcgcagcgacgctgtcccgcgagtgcactcctcgttacattgtgaagtgatatacagtataaacacggattacaacaacgcttatctccacaacatactgaactaatattaattaaaaatggcgacgtcaggagggaaacggcgggaagagggcagcgataactccgatgatgagcttacaccgctcgctaacgatatttatggcggaagccaaaggacagtacaagaaacgaaaggatgggacgtgttccgggagtttccaccgaagcaggacagtgggtctatggagactcagaaatgtttggagttcacagtgcggttgctgaaggtgacggcatatctagtcgtcttcattgcggtcctcgggtccggagtcgtagcaaagggcagcacgctctttatgacatcacagctaaaaaaggacaggcggattgcgtattgtaataggaatttaggtagggataaacaatttatagtaagtcttccagacgaggaacgagtggcttggatgtgggctattttggctgcgttcgccataccagaaataggaacactcattagatcagtgaggatatgctttttcaaaacttctagacgaccgactagcacacaattcgctgtgattttcatagcggagacgttgcatacgataggaatgggtctcctattctttttgatcctaccagaactggacgtggtcaaaggagcaatgattacgaactgcctttgcataattcctgccgttttgggcttgctctcacgcaactccagagattcgaaacggttcataaaagtgattgtggacatggcggcaatagttgcgcaagtcactggattcattgtatggccactattagagaataaacctgtactatggttgataccagtcgcatcactatgcatatcccttggatggtgggaaaactatgtcacacgtcagagtccgataggtataatcaaaagccttggcagattaaaagatgaattaaccttcactcgctactacacgtaccgttttatatctgtctggaaaatcttggtcttcctcatgtgcattctcttcagcatttggctcgaaggtgacgagcctgccatgtttttccaactgttcaatgccggttttggaccacacagtatcgttgtcgaagaggtacaaattcaattaggcgggaccgtcattcctgatttagctaatgttactttaaccggagactcagttgaggtcgcagctgcttacaaatccgcattctacgtgatgcttatccaaatatttgcagcgtatatctgctacatatttggaaagttcgcttgtaagatcctcatccaaggcttcagttacgcgttccccatcaatctcgtcattccattggtggtcaacttgttgattgccgcgtgtggtatcagaaatggtgacaattgctatttccatgggacagttcccgattatctttacttcgagagtccaccagtgtttacgctaagcgatttcatatctcgtcaaatggcatggatatggctactatggctattgtcgcaaacatggatcaccatacacatctggacaccaaaagctgaacgtttggcctctacggagaagttattcgtgatgccaatgtacaacggtttacttattgatcagagtatggccttaaacagaaagaggaatgatcaaagagatgttaagactgaggacctcgcagaaatagaaaaagaaaaaggcgacgaatactatgaaactatatcagttcacacggataacactgggtcttctccaaaagctattaagtcatcagatcagatcaccaggatatatgcatgcgctactatgtggcacgaaactaaagacgagatgatggagttcttgaagtccattcttcggttagacgaggatcagtgcgctcggcgtgtagctcaaaagtatttacgagtcgttgaccctgattactatgaattcgaaacacatatcttcttagacgacgccttcgaaatatcagatcacagtgacgatgattctcaggtgaatcgattcgtaaaactgcttgttgacactatcgatgaagcggcttccgaggtacatcagacgaacattcgtattcgaccacctaagaagtatcccgcgccttacggaggacgattgacgtgggtactgccaggaaagacgaagatgatttgtcacttgaaggataaggcaaagattcgtcacaggaaacgttggtctcaggtgatgtacatgtactacctactcggtcaccgactaatggagctgccaatatctgtggatcgtaaagaagttatggctgagaacacctatctgctgaccctggacggagacatcgatttccaacctcatgctgtacgtttgcttatcgatttgatgaagaagaacaagaatctgggagctgcttgcggtcgtattcatcccgtaggctctggccctatggtgtggtatcaaatgttcgagtatgccattggtcattggctgcaaaaggcaactgaacacatgattggctgtgtactgtgtagccctggctgcttctccctcttcagaggaaaggctttgatggacgacaacgtaatgaagaagtatacattgaggtctgatgaagctcggcattacgtacagtacgatcaaggggaagatcgatggttatgtacgctgttacttcaacgaggttaccgtgtagagtactcagctgcctccgacgcctacactcactgtcccgaaggttttaacgagttctacaaccaacgtcgtcgttgggtgccttccaccatcgccaacattatggacttgcttgccgattgcaaacacaccatcaagattaacgataacatctccagtccttatatcgcataccagatgatgttgatgggtggtacaatcttgggtcccggaactatattccttatgttggtgggtgccttcgtggccgctttccgtattgacaactggacttctttcgaatataacttgtatcccattttgatcttcatgtttgtatgttttacgatgaaatccgaaattcaattgctcgtggctcagatattatcgacggcatacgccatgattatgatggcttttatagtcggtaccgcgcttcagttaggcgaggacggtatcggatctccttcggctatatttttgatatcactttcgagttcgttcttcatagccgcttgcttgcatccgcaggagttctggtgtattgtaccgggaattatttatcttttatctataccctctatgtacttgcttttgattttatattcgattataaatcttaacgtagtatcttggggtactcgagaagtagctgttaagaagacgaagaaggaaatcgaagcagaaaagaaagaagcagaattagcaaaaaaatcggcaaaacagaagtctttgttaggtttccttcaaggagtaaacagcaatgaagaagaaggatctatagaattctcgttcgccggtctattcaagtgtctgttatgcacgcatccaaaaggaaacgaagagaaagtgcaactcttgcatattgcatctactctagagaagttggaaaagaaattagaaactgttgagagggctgttgatcctcacggcattagcagaggacgtaaactgtcggttggaccaagaggtagcaccactggagatcatggtttggacgctctagctgaaggaccagaagaggataacgactcagattctgaaactgacacactttctactgtgccaagagaaaagagagatgatctcataaacccatactggattgaggatcctgagttgaaaaagggtgaagtagactttttgagtcccgccgaattatctttctggaaagatctcattgacaaatatttataccctattgatgctaacaaggaggagcaggcccgtatatccaaggatctgaaagaattgagagactcgtctgttttttctttctttatggtcaatgctctctttgtattgattgtattcttgctacaactgaacaaggacaaccttcacattaagtggcccttcggagttaaaactaacataacatacgatgaggttactcaagaggtgttaatatcaaaggaatatctgcaactggagcctattggtttagtgtttgtattcttcttcgccttgatcctggtgatacagttctccgccatgttgttccatagatttggaaccctttcacacatattagcgtcgacagaactgaactggttctgttctaagaagtccgacgacttgtctcaagacgcactattagataagaatgcaatagcaatagtaaaagacctgcagaaattgaatggtctggacgacgattatgacaatgactcgggctcgggtcctcataacgtcggcagaagaaagactattcacaatttggagaaggcgagacagaagaagaggaatataggcacactggatgtggccttcaagaagagattcttcaatatgaacgccaacgatggaccaggtacaccagttctaaatcgtaagatgacgttgagaagggaaacgctaaaggctttagagacgagaaggaattcagtgatggcggaaagaagaaaatcccagatgcaaacacttggtgccaataatgaatatggagtgacaggaatgctcaataataacttaggtgtcgggccgcggcacaggacatctaatgccaacatatcagtgaaagatgttttcggcgagccaaacggaggtcaagtcaaccgaggctacgaaaccaccataggcgacgaagatgacacaaactcaatgagattacaacctagacaaaaccaagtttccttccagggtagattctaaaagagttgccaaactaagtgcctaggttaaacaaatgtagatactagaaatatagactgtaaaattttttacaatgaagaatctcagcaaatgtttgcgggaatcatgtattgcttgtgatatatacttttttttaggtcgtgacagcaatgtgctgtcattaaataccaacatcggacaatttacagctttattgtaagataaaacatacgaatttacactgccacttaactttacattattgatctttttatacttatttaaaataatatcttttgtattaaaagatttttgttttagtttttatgaaagtagacatcgaattagtgttgtatgtttttaatgggg

SEQ ID NO: 25 - RNA, 543 nt, Spodoptera littoralis
cuaauacgacucacuauagggagaacuugggcuuggagaugaugacgcuaauauugaagaugacuuuaucaccuggaaagaaaaguucuggccagcuguaugugagaaauucaauauugagagcacuggugaagaagaguugauucgucaguuccgucuuguuacucacggaccugaugacauacaaccuaacaacauauuuacuggagaaauugccagauuacacuccuuacaaguccagaggccaccuuaugaugccaagaauccauuccuugcucaaaucacaguuaauagagaauuacauaaggguggagauaggucuuguauccaugucgaauuggauauuucagacuccaaaaugcgauaugaagcaggugaucauguggcuguguacccaauaaaugacucuaaccuuguagaucgucuaggacaauuaacaggggccaaccuugacgagaucuucucucucaucaacacugaccaggaaagcagcaaaaagcauccuuucccuugcccaacucucccuauagugagucguauuag

SEQ ID NO: 26 - RNA, 533 nt, Spodoptera littoralis
cuaauacgacucacuauagggagaccaaccuugacgagaucuucucucucaucaacacugaccaggaaagcagcaaaaagcauccuuucccuugcccaaccuccuaucgcacugcauuaucacacuauguugagauuacugcauugccccguacucacauauuaagagaguugguugaauacuguacagaugaagaagacaaaaagaaauugaugcucauggcaacuaauucucaagagggcaaggccauguaccaaucauuuauuguagaggcuugcagaaauauugugcacaucuuggaagauguaccaucuuguaaaccuccacuggaccacuugugugaacuuuuaccucgccuacaaccaagauacuacuccaucucauccaguccuaagauguauccagagacagugcauauuacugcagucguuguucaauauaaaacaccuacgggucgcgucaacaaagguguuacgacaacaugguuagcagauaacaaacccgaacccucucccuauagugagucguauuag

SEQ ID NO: 27 - DNA, 44 bp, Spodoptera littoralis
ctaatacgactcactatagggagaacttgggcttggagatgatg

SEQ ID NO: 28 - DNA, 44 bp, Spodoptera littoralis
ctaatacgactcactatagggagagttgggcaagggaaaggatg

SEQ ID NO: 29 - DNA, 44 bp, Spodoptera littoralis
ctaatacgactcactatagggagaccaaccttgacgagatcttc

SEQ ID NO: 30 - DNA, 44 bp, Spodoptera littoralis
ctaatacgactcactatagggagagggttcgggtttgttatctg

SEQ ID NO: 31 - RNA, 525 nt, Spodoptera littoralis
cuaauacgacucacuauagggagaccggaaagcccauugacaagggucccccaauccucgccgaggacuucuuggacauccagggacagcccaucaacccauggucccguaucuaccccgaggagaugauccagacugguaucuccgcuaucgacgugaugaacuccauugcucguggucagaagauccccaucuucucugccgcuggucugccccacaaugaaauugccgcccagaucuguagacaggccggucuuguuaagauccccggcaaaucaguguuggaugaccacgaggacaacuucgccaucguauucgcagcuaugggugugaacauggaaaccgcccgguucuucaaacaggacuucgaagagaacgguucuauggagaacgugugccuguucuugaacuuggccaaugaccccacuauugagagaauuaucacaccccgucuugcuuugacugcugccgaguucuuggccuaccagugcgagaaacacgucucccuauagugagucguauuag

SEQ ID NO: 32 - DNA, 45 bp, Spodoptera littoralis
ctaatacgactcactatagggagaccggaaagcccattgacaagg

SEQ ID NO: 33 - DNA, 45 bp, Spodoptera littoralis
ctaatacgactcactatagggagacgtgtttctcgcactggtagg

SEQ ID NO: 34 - RNA, 524 nt, Spodoptera littoralis
cuaauacgacucacuauagggagauucgugcgcaagcucaacgguagugccagcagcgacacggguaguucgggccaggacgaauguggggcccgcgccacucccuccgguaccucuccgccacguauggccggucccgugcacccacgauaugcgucugaagccgcacgacuacguagcuuuaaagacuggccacgaugcaugcggcaaaaaccugaagaacucgcagaggcuggcuuuuuuuacacuggucagggagacaaaaccaaguguuuuuacugcgaugguggauuaaaagauugggagaaccaugacguacccugggaacaacaugcacggugguuugaccguugcgccuacgugcaauuggugaagggucgagaauacguucaaaaggugauuucugaggcuugugagguauccgcaucggaagcagaacgugauguugcucccucacgaacuaccagcgaguccagcgcgccaguugagacgccggagaaucucccuauagugagucguauuag

SEQ ID NO: 35 - DNA, 44 bp, Spodoptera littoralis
ctaatacgactcactatagggagattcgtgcgcaagctcaacgg

SEQ ID NO: 36 - DNA, 44 bp, Spodoptera littoralis
ctaatacgactcactatagggagattctccggcgtctcaactgg

SEQ ID NO: 37 - RNA, 513 nt, Spodoptera exigua
cuaauacgacucacuauagggagauauucaucccguaggcucuggcccuauggugugguaucaaauguucgaguaugccauuggucauuggcugcaaaaggcaacugaacacaugauuggcuguguacuguguagcccuggcugcuucucccucuucagaggaaaggcuuugauggacgacaacguaaugaagaaguauacauugaggucugaugaagcucggcauuacguacaguacgaucaaggggaagaucgaugguuauguacgcuguuacuucaacgagguuaccguguagaguacucagcugccuccgacgccuacacucacugucccgaagguuuuaacgaguucuacaaccaacgucgucguugggugccuuccaccaucgccaacauuauggacuugcuugccgauugcaaacacaccaucaagauuaacgauaacaucuccaguccuuauaucgcauaccagaugauguugauggguggucucccuauagugagucguauuag

SEQ ID NO: 38 - RNA, 713 nt, Spodoptera exigua
cuaauacgacucacuauagggagacugcaacuggagccuauugguuuaguguuuguauucuucuucgccuugauccuggugauacaguucuccgccauguuguuccauagauuuggaacccuuucacacauauuagcgucgacagaacugaacugguucuguucuaagaaguccgacgacuugucucaagacgcacuauuagauaagaaugcaauagcaauaguaaaagaccugcagaaauugaauggucuggacgacgauuaugacaaugacucgggcucggguccucauaacgucggcagaagaaagacuauucacaauuuggagaaggcgagacagaagaagaggaauauaggcacacuggauguggccuucaagaagagauucuucaauaugaacgccaacgauggaccagguacaccaguucuaaaucguaagaugacguugagaagggaaacgcuaaaggcuuuagagacgagaaggaauucagugauggcggaaagaagaaaaucccagaugcaaacacuuggugccaauaaugaauauggagugacaggaaugcucaauaauaacuuaggugucgggccgcggcacaggacaucuaaugccaacauaucagugaaagauguuuucggcgagccaaacggaggucaagucaaccgaggcuacgaaaccaccauaggcgacgaucucccuauagugagucguauuag

SEQ ID NO: 39 - DNA, 44 bp, Spodoptera exigua
ctaatacgactcactatagggagatattcatcccgtaggctctg

SEQ ID NO: 40 - DNA, 44 bp, Spodoptera exigua
ctaatacgactcactatagggagaccacccatcaacatcatctg

SEQ ID NO: 41 - DNA, 44 bp, Spodoptera exigua
ctaatacgactcactatagggagactgcaactggagcctattgg

SEQ ID NO: 42 - DNA, 44 bp, Spodoptera exigua
ctaatacgactcactatagggagatcgtcgcctatggtggtttc

SEQ ID NO: 43 - RNA, 495 nt, Zea mays
uaauacgacucacuauagggagauuggcgagcuuaggauugaggaucguuuacaguggaaagaacacucuaugauauucgccaugccaaacaagccaggagaauucagccgguuugauuucccagaaacuuugccagcaccuauaaaugggauaugggccauauugagaaacaaugaaaugcuuaccuggcccgagaaggugaaguuugcaaucggacuucugccagcaaugguugguggucaaccuuauguugaagcucaagauggcuuaaccguuucagaauggaugaaaaagcaggguguuccugaucgggugaacgaugagguuuuuauugcaauguccaaggcacucaauuucauaaauccugaugagcuaucuaugcagugcauuuugauugcuuugaaccgauuucuucaggagaagcaugguucuaaaauggcauucuuggaugguaauccgccugaaaggcuaucucccuauagugagucguauua

SEQ ID NO: 44 - RNA, 593 nt, Zea mays
uaauacgacucacuauagggugaucgggugaacgaugagguuuuuauugcaauguccaaggcacucaauuucauaaauccugaugagcuaucuaugcagugcauuuugauugcuuugaaccgauuucuucaggagaagcaugguucuaaaauggcauucuuggaugguaauccgccugaaaggcuaugcaugccuauuguugaucacauucggucuagggguggagagguccgccugaaucucguauuaaaaagauagagcugaauccugauggaacuguaaaacacuucgcacuuagugauggaacucagauaacuggagaugcuuauguuugugcaacaccagucgauaucuucaagcuucuuguaccucaagaguggagugaaauuacuuauuucaagaaacuggagaaguuggugggaguuccuguuaucaauguucauauaugguuugacagaaaacugaacaacacauaugaccaccuucuuuucagcaggaguucacuuuuaagugucuaugcagacaugucaguaaccugcaaggaauacuaugacccaaaccguucaaugcuggcccuauagugagucguauua

SEQ ID NO: 45 - DNA, 20 bp, artificial Sequence
  polynucleotide sequence or in vitro generated dsRNA
gattgctggagcaggattag

SEQ ID NO: 46 - DNA, 20 bp, artificial Sequence
  polynucleotide sequence or in vitro generated dsRNA
cccttgcctcaagcaatatg

SEQ ID NO: 47 - DNA, 21 bp, artificial Sequence
  polynucleotide sequence or in vitro generated dsRNA
accacttcgaccgccactact

SEQ ID NO: 48 - DNA, 19 bp, artificial Sequence
  polynucleotide sequence or in vitro generated dsRNA
acgcctaagcctgctggtt

SEQ ID NO: 49 - DNA, 20 bp, artificial Sequence
  polynucleotide sequence or in vitro generated dsRNA
accggcatcagctcagtctc

SEQ ID NO: 50 - DNA, 20 bp, artificial Sequence
  polynucleotide sequence or in vitro generated dsRNA
tgctgttctctgggcacagg

SEQ ID NO: 51 - DNA, 20 bp, artificial Sequence
  polynucleotide sequence or in vitro generated dsRNA
tcccctcagatattaacaac

SEQ ID NO: 52 - DNA, 22 bp, artificial Sequence
  polynucleotide sequence or in vitro generated dsRNA
aggaggaaaggcagcttctgtg

SEQ ID NO: 53 - DNA, 20 bp, artificial Sequence
  polynucleotide sequence or in vitro generated dsRNA
gtgactcgtcaccaacaaag

SEQ ID NO: 54 - DNA, 20 bp, artificial Sequence
  polynucleotide sequence or in vitro generated dsRNA
tgtgttgtccgttgagactg

SEQ ID NO: 55 - DNA, 20 bp, artificial Sequence
  polynucleotide sequence or in vitro generated dsRNA
tcggaagccgtaccttcgtg

SEQ ID NO: 56 - DNA, 20 bp, artificial Sequence
  polynucleotide sequence or in vitro generated dsRNA
cctggagctgctgctttgtg

SEQ ID NO: 57 - DNA, 20 bp, artificial Sequence
  polynucleotide sequence or in vitro generated dsRNA
taccaggcgtcgagtggttc

SEQ ID NO: 58 - DNA, 20 bp, artificial Sequence
  polynucleotide sequence or in vitro generated dsRNA
gaagagggcgtgcaaatggg

SEQ ID NO: 59 - DNA, 20 bp, artificial Sequence
  polynucleotide sequence or in vitro generated dsRNA
ctattgcgtgtgctccaaac

SEQ ID NO: 60 - DNA, 20 bp, artificial Sequence
  polynucleotide sequence or in vitro generated dsRNA
acatgaggaggaaccaaagg

SEQ ID NO: 61 - RNA, 490 nt, artificial Sequence
  polynucleotide sequence or in vitro generated dsRNA
cuaauacgacucacuauagggagaggcucaagaaccaguuuauguuaaugcuaagcaguaucgaaggauccugcagcgaagacagucacgugcuaaagcagaacuugaaaagaagcaaauaaaggguagaaagccauaucuucacgagucucgacaucagcaugcacugaggaggguaagggccucggguggacguuuugccaaaaagacagaugcuucuaaggguacugguucugugaguucaucggguucugaaccuuugcaguucaaugcugcugauauucaaaagaggaaugaaaauggaagguuggccgagcuucagcagucuuauucaaaugguagcaguuauggcaaucaaaguagcuuucaagaauccaaggaugaguaccaguuugcuaaaagcagggaaggagguuuuuuugucaaguaauuggagauacguucauguguaaacuagcucuugcccucucccuauagugagucguauuag

SEQ ID NO: 62 - RNA, 497 nt, artificial Sequence
  polynucleotide sequence or in vitro generated dsRNA
cuaauacgacucacuauagggagagcaguuauggcaaucaaaguagcuuucaagaauccaaggaugaguaccaguuugcuaaaagcagggaaggagguuuuuuugucaaguaauuggagauacguucauguguaaacuagcucuugcccugcaacgaggguagaguaugagcaagaggaguuuacagggauuguuucauuucuuggcuuuucaagauaggcggcaauucauucuuggcuuuuuacuuuaguguuaaagggagcaacagaggugacgaggguaucaguguugcagcauuugcuuggagauuacaucuucccuuauguacagagauggaugaacuuagaacuaggauuagaaaguuuuucaguaaguuuauguuuggccaguuacuguaguuuuaguuuaggagaccauguaaaaagguuguuaguuuugcaaaaggaucuuuuuucuuucccuaauuggugcauucucccuauagugagucguauuag

SEQ ID NO: 63 - DNA, 20 bp, artificial Sequence
  polynucleotide sequence or in vitro generated dsRNA
cgagtcgggatactggaagg

SEQ ID NO: 64 - DNA, 20 bp, artificial Sequence
  polynucleotide sequence or in vitro generated dsRNA
cttcttcatgccgacgaggg

SEQ ID NO: 65 - DNA, 20 bp, artificial Sequence
  polynucleotide sequence or in vitro generated dsRNA
acgatgggcgagaaggagtg

SEQ ID NO: 66 - DNA, 20 bp, artificial Sequence
  polynucleotide sequence or in vitro generated dsRNA
tcagtcccgtcgggtacttg

SEQ ID NO: 67 - DNA, 20 bp, artificial Sequence
  polynucleotide sequence or in vitro generated dsRNA
agggtcacatcccgaactac

SEQ ID NO: 68 - DNA, 20 bp, artificial Sequence
  polynucleotide sequence or in vitro generated dsRNA
acctcgtcagtctccacatc

SEQ ID NO: 69 - DNA, 20 bp, artificial Sequence
  polynucleotide sequence or in vitro generated dsRNA
gttggattcgagcttccttc

SEQ ID NO: 70 - DNA, 20 bp, artificial Sequence
  polynucleotide sequence or in vitro generated dsRNA
tgctgctgctcactagctac

SEQ ID NO: 71 - RNA, 490 nt, artificial Sequence
  polynucleotide sequence or in vitro generated dsRNA
cuaauacgacucacuauagggagacaguccguuggccuaguuccuauuggagaucugugaagguugguugggaugaaucaacugcaggggaaagaccaccaagaguuucuuuaugggaaauugaaccauugacaaccuuuccaauguauccaucucuguucccacugagaguuaagcauccuugguauucaggaguugcuucccugcaugaugacagcaaugcuuuaauguggcugagaggaguugcuggugagggagguuuucagucucugaacuuucagucaccugguauuggcuccuggggacaacagaggcuccauccauccuuacugagcagcgaucacgaucaguaccaagcaguaguugcugcugcugcugcuucccaaucuggugguuacuuaaaacagcaauucuugcaccuucagcaaccuaugcaguccccucaagaacacugcaaccucaacccucucccuauagugagucguauuag

SEQ ID NO: 72 - DNA, 20 bp, artificial Sequence
  polynucleotide sequence or in vitro generated dsRNA
ctcagccatgggatactacc

SEQ ID NO: 73 - DNA, 20 bp, artificial Sequence
  polynucleotide sequence or in vitro generated dsRNA
gctggccgttgacgacattg

SEQ ID NO: 74 - DNA, 18 bp, artificial Sequence
  polynucleotide sequence or in vitro generated dsRNA
acctcaggtggatgtctc

SEQ ID NO: 75 - DNA, 18 bp, artificial Sequence
  polynucleotide sequence or in vitro generated dsRNA
tgctggtgctttgggtag

SEQ ID NO: 76 - DNA, 530 bp, Zea mays
taccatgcgatccttaggaggaggcagacacgtgctaaactggaggcgcaaaacaagatggtgaaaggtcggaagccgtaccttcgtgagtctcgacaccgtcatgccatgaagcgggcccgtggctcaggagggcggttcctcaacacaaagcagcagctccaggagcagaaccagcagtaccaggcgtcgagtggttcaatgtgctcaaagaccattggcgacagcgtaatctcccaaagtggccccatttgcacgccctcttctgacgctgcaggtgcttcagcagccagccaggaccgcggctgcttgccctcggttggcttccgccccacagccaacttcagtgagcaaggtggaggcggctcgaagctggtcgtgaacggcatgcagcagcgtgtttccaccataaggtgaagagaagtgggcacgacaccattcccaggcgcgcactgcctgtggcaactcatccttggcttttgaaactatgaatatgcaatggacatgtagctttgagttcctcagaataa

SEQ ID NO: 77 - DNA, 40 bp, artificial Sequence
  polynucleotide sequence or in vitro generated dsRNA
taatacgactcactatagggccgcatgccattgtccatcc

SEQ ID NO: 78 - DNA, 40 bp, artificial Sequence
  polynucleotide sequence or in vitro generated dsRNA
taatacgactcactatagggtgcatgccgttcacgaccag

SEQ ID NO: 79 - DNA, 40 bp, artificial Sequence
  polynucleotide sequence or in vitro generated dsRNA
taatacgactcactatagggcaaatagtccggttatgttg

SEQ ID NO: 80 - DNA, 42 bp, artificial Sequence
  polynucleotide sequence or in vitro generated dsRNA
taatacgactcactataggggctacatgtccattgcatattc

SEQ ID NO: 81 - RNA, 936 nt, Oryza sativa
ucaguguuuguccccucagauauuaacaacaaugauaguuguggggagcgggaccauggcacuaagucgguauugucuuuggggaacacagaagcugccuuuccuccuucaaaguucgauuacaaccagccuuuugcauguguuucuuauccauaugguacugauccauauuaugguggaguaucaacaggauacacuucacaugcauuuguucauccucaaauuacuggugcugcaaacucuaggaugccauuggcuguugauccuucuguagaagagcccauauuugucaaugcaaagcaauacaaugcgauccuuagaagaaggcaaacgcgugcaaaauuggaggcccaaaauaaggcggugaaaggucggaagccuuaccuccaugaaucucgacaucaucaugcuaugaagcgagcccguggaucagguggucgguuccuuaccaaaaaggagcugcuggaacagcagcagcagcagcagcagcagaagccaccaccggcaucagcucagucuccaacagguagagccagaacgagcggcggugccguuguccuuggcaagaaccugugcccagagaacagcacauccugcucgccaucgacaccgacaggcuccgagaucuccagcaucucauuugggggcggcaugcuggcucaccaagagcacaucagcuucgcauccgcugaucgccaccccacaaugaaccagaaccaccguguccccgucaugaggugaaaaccucgggaucgcgggacacgggcgguucugguuuacccucacuggcgcacuccggugugcccguggcaauucauccuuggcuuaugaaguaucuaccugauaauagucugcugucaguuuauaugcaaugcaaccucugucagauaaacucuuauaguuuguuuuauuguaagcuaugacugaacgaacugu

SEQ ID NO: 82 - DNA, 43 bp, artificial Sequence
  polynucleotide sequence or in vitro generated dsRNA
taatacgactcactatagggctgcctttcctccttcaaagttc

SEQ ID NO: 83 - DNA, 40 bp, artificial Sequence
  polynucleotide sequence or in vitro generated dsRNA
taatacgactcactatagggtgctgttctctgggcacagg

SEQ ID NO: 84 - DNA, 41 bp, artificial Sequence
  polynucleotide sequence or in vitro generated dsRNA
taatacgactcactatagggcattggctgttgatccttctg

SEQ ID NO: 85 - DNA, 40 bp, artificial Sequence
  polynucleotide sequence or in vitro generated dsRNA
taatacgactcactatagggttcgttcagtcatagcttac

SEQ ID NO: 86 - RNA, 512 nt, Oryza sativa
caugguggcucagcggcuggggcaccaaugcuccaccacccagccuuugagcucaccucagguggaugucucgcgggagucgccaccgacuccagcugugcucucucucuucugucaacucagccaugggauacuacccaaagcaccagcagccacaaccgguccccgccaaugucgucaacggccagcgccuucggaggcggcaacaacccggugucgcccucggucauggcaagcaacuacauggcggcgagccccggcuggaacagcuccagccggggccaugacggcgccaggaacgugcaccugccgccaccgcacgggguugugcugaacgaggucccuccgggcucuguccaccacggccauuucuccggcgagcucgagcucgcacugcagggaggugccccguccaaccggccggaagccaagcauggcuccggcagcggcgccuucagccacuccaccaaugccaugaacuggucucuguagagaccauugaucaucuucuu

SEQ ID NO: 87 - DNA, 40 bp, artificial Sequence
  polynucleotide sequence or in vitro generated dsRNA
taatacgactcactatagggtcacctcaggtggatgtctc

SEQ ID NO: 88 - DNA, 40 bp, artificial Sequence
  polynucleotide sequence or in vitro generated dsRNA
taatacgactcactatagggcattggtggagtggctgaag

SEQ ID NO: 89 - DNA, 44 bp, artificial Sequence
  polynucleotide sequence or in vitro generated dsRNA
taatacgactcactatagggccaatgctccaccacccagccttt

SEQ ID NO: 90 - DNA, 43 bp, artificial Sequence
  polynucleotide sequence or in vitro generated dsRNA
taatacgactcactatagggagttcatggcattggtggagtgg

SEQ ID NO: 91 - RNA, 840 nt, Zea mays
auggaaggaaacgguggcgcgggcggcgguagcggaagcgcggcaccgcccugggaucucgccaugcacugggcacccgccguagugucguccuacccgccgcagcccuuggagcugcagcagcaggagcuuaccugccucaagcuggggaagcggcccgccugcugcugggcaggggcgccgggcaaccaagcggcgcagguccacggcaauggcggcgcugguggcgcagcugcugaggguaagaggaaggacaaggcgccugccgcggcggccgugacgaggugccagguggaggggugccaccugucgcuggcggacgccaaggaguaccaccggcggcacaaggugugcgaggcgcacuccaagucgccccgggucgucguccucggcgccgagcagcgcuucugccagcagugcagccgguuccacgcgaucucggaguucgacgacgcgaagcggagcugccgacggcgucuggccgggcacaacgagcggcggcggaagagcaacgccagcgaggccauggcaagaggcgucgcgcacccacacggagugacggcuuucggccacggcggcuuccugcccucgcgcggccucguccccgcagggucguccccggcggcggcuggugcucucucucuucugucaucggccagaggcagcguggcgggcgccagcgggcccuggcuggucacggcggcgcgggaggacaucccggcgcgcuccagcgcggcgcucgacgaccuuaucgccgagaaccgcgccgccgcgcuccucgcgcggcaguacuucgucuccgaccgcucgccggcgcccagacgggauuucgucgccucu

SEQ ID NO: 92 - DNA, 40 bp, artificial Sequence
  polynucleotide sequence or in vitro generated dsRNA
taatacgactcactatagggcgccgtagtgtcgtcctacc

SEQ ID NO: 93 - DNA, 40 bp, artificial Sequence
  polynucleotide sequence or in vitro generated dsRNA
taatacgactcactatagggaaagccgtcactccgtgtgg

SEQ ID NO: 94 - DNA, 38 bp, artificial Sequence
  polynucleotide sequence or in vitro generated dsRNA
taatacgactcactatagggcgcaggtccacggcaatg

SEQ ID NO: 95 - DNA, 41 bp, artificial Sequence
  polynucleotide sequence or in vitro generated dsRNA
taatacgactcactatagggcggtcggagacgaagtactgc

SEQ ID NO: 96 - RNA, 800 nt, Oryza sativa
augagcgggaugaauucgcugagcaugguggaggcgaggcugccgccgggguucagguuccacccgcgagacgacgagcucgugcuggacuaccuggaaaggaagcuccucgacggcggcgugggcggcgccgcggcggcggcggcggcggucaccaucuacggcugcccggugauggucgacgucgaucucaacaagugcgagccaugggaccuuccugagaucgcuugcguugguggcaaggagugguacuucuauagccuuagggauaggaaguaugcaacuggccaacgaacaaauagagcaaccgaaucgggcuacuggaaggccacaggaaaagaucgcccaauaagccggaaaggauugcucgucgguaugcgaaaaacccugguguucuacaaagguagagccccuaaggggaagaagaccgagugggucaugcaugaauuccgcaaagaaggacaaggggauccgaugaaguugccucucaaggaggacugggucuuguguagagucuucuacaagaguaggacaaccauugccaagcugccaacggaggguagcuacaacaauauugacaguguggccacaacuucacugccuccccucacugacaacuacauugcauuugaucagccugguucaaugcaaaaccuagaggguuaugagcaagugcccugcuucuccaauaaucccucucaacagccaucgucgucgaugaauguuccguugacaucggccaugguugaucaagagcaaaacaauauggguagggcgaucaaggaugugcugagccaauu

SEQ ID NO: 97 - DNA, 41 bp, artificial Sequence
  polynucleotide sequence or in vitro generated dsRNA
taatacgactcactatagggttcaggttccacccgcgagac

SEQ ID NO: 98 - DNA, 41 bp, artificial Sequence
  polynucleotide sequence or in vitro generated dsRNA
taatacgactcactatagggccgttggcagcttggcaatgg

SEQ ID NO: 99 - DNA, 41 bp, artificial Sequence
  polynucleotide sequence or in vitro generated dsRNA
taatacgactcactatagggcgtgctggactacctggaaag

SEQ ID NO: 100 - DNA, 40 bp, artificial Sequence
  polynucleotide sequence or in vitro generated dsRNA
taatacgactcactatagggcaaccatggccgatgtcaac

SEQ ID NO: 101 - DNA, 799 bp, Zea mays
atggagcacgacgtgcaccaccagcaggccatggagctgccgccggggttccgattccaccccaccgacgaggagctcatcacgcactacctcgccaggaaggccgccgacgcccgcttcgccccgcgcgccgtcggcgaggccgacctcaacaagtgcgagccatgggacctgccatcccgggcgacgatgggcgagaaggagtggtacttcttctgcgtcaaggaccgcaagtacccgacgggactgaggacgaaccgggccaccgagtcgggatactggaaggcgacgggcaaggacagggagatcttcaggagcaaggccctcgtcggcatgaagaagacgctcgtcttctacacggggagggcgcccaggggaggcaagaccggctgggtcatgcacgagtaccgcctccacggcaagcacgccagcagcagccgcctcatgccgtcgtcggtcagagctggcgcgtcaaaggacgagtgggtgctgtgcagggtgttcaagaagagcatcgagccgccgccgtcagtgggcaagaggtcgtcggtcgcgtgtacggggatgatgttggtggaggacgtcgtgggaccgccgtccatgtccatggaggacgacctcgccgcgtgcgcgctgcctccgctgatggacgtgtccggcggtggcggcgccaacatggcggcggcgtccatcgagctgctggcgccaccggcaccacacgtgacctgcttctccaacgcgctggagggccagttcttcctgaacccaccctgcctccacccctccacgtcgccgctcc

SEQ ID NO: 102 - DNA, 40 bp, artificial Sequence
  polynucleotide sequence or in vitro generated dsRNA
taatacgactcactatagggccaccgacgaggagctcatc

SEQ ID NO: 103 - DNA, 40 bp, artificial Sequence
  polynucleotide sequence or in vitro generated dsRNA
taatacgactcactatagggcgacgtcctccaccaacatc

SEQ ID NO: 104 - DNA, 39 bp, artificial Sequence
  polynucleotide sequence or in vitro generated dsRNA
taatacgactcactatagggaggccgacctcaacaagtg

SEQ ID NO: 105 - DNA, 42 bp, artificial Sequence
  polynucleotide sequence or in vitro generated dsRNA
taatacgactcactatagggtcaggaagaactggccctccag

SEQ ID NO: 106 - DNA, 20 bp, artificial Sequence
  polynucleotide sequence or in vitro generated dsRNA
cctcaacagtcctggatgtc

SEQ ID NO: 107 - DNA, 20 bp, artificial Sequence
  polynucleotide sequence or in vitro generated dsRNA
cccgtaagttggaagtgatg

SEQ ID NO: 108 - RNA, 506 nt, artificial Sequence
  polynucleotide sequence or in vitro generated dsRNA
cuaauacgacucacuauagggagagcuucuccucccuacaacugugucuaacgucgcuacuacaucaauugaugcugauauauccucuaugccacuagggacuucuggauuuccgaaucccuuguauaguuaugugcaagauucuacugacuuguugcauaauguagggcaagcugaugcacaaacugugccccguacauuugucaagguuuacaaaucagcgucccuugggaggucauuggacaucacucgguucaacagcuaucaugagcugcgacaggaauuagggcagauguucgguaucgaaggguugcuugaagacccucaaagaucaggcuggcagcuuguauuuguugacagggagaaugauguccuucuccuuggagacgauccgugggaggaauuugucaauaauguuugguacaucaaaauucuuucacccgaggaugugcagaaacuggggaaagaggagguuggaucccucucccuauagugagucguauuag

SEQ ID NO: 109 - RNA, 544 nt, artificial Sequence
  polynucleotide sequence or in vitro generated dsRNA
cuaauacgacucacuauagggagaugggagauugagccuuugacuacuuuuccgauguauccaucucuuuuuccucuaaggcuaaagaggccuuucuaucaaggaaccucaucuuaucaggauaguaacaaugaagcuauuaaucgaaugucaugguuaagagggaaugcuggugagcuaggacaucauucaaugaaucuucagucuuuuggcaugcuuccuuggaugcaacagagagucgauucaacaauucucccaaaugauauuaaucagcacuaucaagcuaugcuggcuacuggcuugcaaaguuuugggaguggagauuuacugaaacagcaauuaaugcaguuucagcagccuguccaauaucugcaacaugcaaguacugagaauucaauuuugcaucagcagcagcagcagcagcagcaaauaaugcagcaagcaguucaucagcauaugcugccugcucaaacccaaaugcugucagagaaccuucaaaggcaaucccagcaucaauccaucucccuauagugagucguauuag

SEQ ID NO: 110 - DNA, 20 bp, artificial Sequence
  polynucleotide sequence or in vitro generated dsRNA
gaggcaccttgtgttgattg

SEQ ID NO: 111 - DNA, 20 bp, artificial Sequence
  polynucleotide sequence or in vitro generated dsRNA
caaagccacggttcttaagc

SEQ ID NO: 112 - RNA, 511 nt, artificial Sequence
  polynucleotide sequence or in vitro generated dsRNA
cuaauacgacucacuauagggagauccagguccaaugaaacaaccuuauguuccuccucacuauguaucugcccccggcaccaccacggcgcgguggucgacuggucuuugucauuguuuugaugacccugcuaacuguuuaguuacuaguguuugcccuuguaucaccuuuggacagauuucugaaauacuaaacaaaggaacaacuucaugugggaguagaggugcauuauauuguuugcugggauugacaggauugccuagccuauauuccugcuucuacaggucuaaaaugagggggcaauaugaucuggaagaggcaccuuguguugauugucuuguacauguauucugugaaccuugugcucuuugccaagaauacagagagcuuaagaaccguggcuuugauaugggaauaggguggcaagcuaauauggauagacaaagccgaggaguuaccaugcccccuuaucaugcaggcaugaccucucccuauagugagucguauuag

SEQ ID NO: 113 - RNA, 513 nt, artificial Sequence
  polynucleotide sequence or in vitro generated dsRNA
cuaauacgacucacuauagggagaagcuccugaacccaucauugaagaaccagugcuuagccuugauccaguugcagcagccauuucgaugaugucuggcagugagaacguaauggaugaaacuauagagguugcagauaucagcgacauucagaaugacucucuuuuaagcgaaguauuauacgagugcgagaaggaacucauggagaaguccgcaaucgaagagacuauuucugaacugcuggacgucaagauuccuaugcugcaaguggaagaguucccuagggaaacccaaguacaacuaccggccauggagaaggagaagccaucaguuccugaauguuguucacuccagaaaagugucaguucugggugccucaacucagcugauuggaucaauggaccagccaggccaaacuuccuggacuuccaaggauuggacuuugagacagcguuuggguugaggagggcauacagcgaaggagacauucucccuauagugagucguauuag

SEQ ID NO: 114 - RNA, 524 nt, artificial Sequence
  polynucleotide sequence or in vitro generated dsRNA
cuaauacgacucacuauagggagacauggagaaguccgcaaucgaagagacuauuucugaacugcuggacgucaagauuccuaugcugcaaguggaagaguucccuagggaaacccaaguacaacuaccggccauggagaaggagaagccaucaguuccugaauguuguucacuccagaaaagugucaguucugggugccucaacucagcugauuggaucaauggaccagccaggccaaacuuccuggacuuccaaggauuggacuuugagacagcguuuggguugaggagggcauacagcgaaggagacauucagaaucuuggagcuagcaccccucgacccgggaacucaggaaacgcucaauuagcaucuugcgagaggcuuguaaccaucagugaccugaaaucugaagaaaggaagcagaagcuaucuagguacagaaagaagaaggugaagagaaacuuuggcagaaagaucaaguaugcuugcaggaaggcucucucccuauagugagucguauuag

SEQ ID NO: 115 - DNA, 20 bp, artificial Sequence
  polynucleotide sequence or in vitro generated dsRNA
gtgactcgtcaccaacaaag

SEQ ID NO: 116 - DNA, 20 bp, artificial Sequence
  polynucleotide sequence or in vitro generated dsRNA
tgtgttgtccgttgagactg

SEQ ID NO: 117 - DNA, 20 bp, artificial Sequence
  polynucleotide sequence or in vitro generated dsRNA
cagttcgcgcacaccattcg

SEQ ID NO: 118 - DNA, 20 bp, artificial Sequence
  polynucleotide sequence or in vitro generated dsRNA
gcagcatgaacggctccaag

SEQ ID NO: 119 - DNA, 20 bp, artificial Sequence
  polynucleotide sequence or in vitro generated dsRNA
tccgcaatgccgtgtgcatc

SEQ ID NO: 120 - DNA, 20 bp, artificial Sequence
  polynucleotide sequence or in vitro generated dsRNA
gcggcaggaatgctagtgtc

SEQ ID NO: 121 - RNA, 543 nt, artificial Sequence
  polynucleotide sequence or in vitro generated dsRNA
cuaauacgacucacuauagggagagcccacuucuacgaguccugccccuaccucaaguucgcccacuucaccgcaaaucaagccauccucgaggcuuucgccggcugccaccgcguccacgucgucgacuucggcaucaagcaggggaugcaauggccagcucuccuccaggcccucgcccuucgucccggcggccccccaucguuccgccucaccggcgucggccccccgcagccggacgagaccgacgccuugcagcagguggguuggaagcuugcccaguucgcgcacaccauucgcgucgacuuccaguaccggggacucgucgccgccacucucgcggacuuggagccguucaugcugcagccggagggcgaggcggacgcgaacgaggagccugaggugaucgccgucaacucgguguucgagcugcaccggcugcucgcgcagcccggcgcgcuggagaagguccugggcacggugcacgcggugcggccaaggaucgucaccgugguagagucucccuauagugagucguauuag

SEQ ID NO: 122 - RNA, 547 nt, artificial Sequence
  polynucleotide sequence or in vitro generated dsRNA
cuaauacgacucacuauagggagaauaucuacaaccgcgacuggcauuauucauguggaacaaaagacuacaaauuacugauggauaaguuucgccuugucuccacggcuuucuuggagcuuggucaagguuaucaagaggcaauugaagaaaucacuaggcuaaugggagcaggaauggcaaaauuuaucugcaaggagguugaaacuguugaugacuacaaugaguacugucacuauguagcagggcuagugggguaugggcuuuccaggcucuuucaugcuggugggacggaagaucuggcuucagauucacuuucaaauucaaugggcuuguuucugcagaaaaucaauauaauuagggauuauuuggaggacauaaacgagauaccaaagucacguauguucuggccucgagaaauauggaguaaauaugucaauaaacucgaggauuugaaauacgaggaaaauucagaaaaggcaguucaguguuugaaugauauggugacuaacgcucugucucaucucccuauagugagucguauuag

SEQ ID NO: 123 - RNA, 455 nt, artificial Sequence
  polynucleotide sequence or in vitro generated dsRNA
cuaauacgacucacuauagggagacgcucugucucaugcugaagacugccuccaauacaugucagcauugaaggaucaugccauuuuccguuuuugugcaauaccucagauaauggcaauugggacaugugcuauuugcuacaauaaugugaaugucuuuagaggaguuguuaagaugaggcgugggcucacugcacgaguaauugaugagacaaacacaaugucagaugucuauacugcuuucuaugaguucucuucgcugauagaaucgaagauugauaauaaugauccaaaugcuucccuaacgcggaaacguguugaugcgauaaagagaaccugcaagucaucuugcucacuaaagagaaggggauacgauuuggagaagucaaaguacaacuccaugcugauaaugguuguacuucuguugguggcucucccuauagugagucguauua

SEQ ID NO: 124 - RNA, 480 nt, Aqueoria victoria
cuaauacgacucacuauagggcgagccaacacuugucacuacuuucucuuaugguguucaaugcuuuucaagauacccagaucauaugaagcggcacgacuucuucaagagcgccaugccugagggauacgugcaggagaggaccaucucuuucaaggacgacgggaacuacaagacacgugcugaagucaaguuugagggagacacccucgucaacaggaucgagcuuaagggaauugauuucaaggaggacggaaacauccucggccacaaguuggaauacaacuacaacucccacaacguauacaucacggcagacaaacaaaagaauggaaucaaagcuaacuucaaaauuagacacaacauugaagauggaagcguucaacuagcagaccauuaucaacaaaauacuccuauuggcgauggcccuguccuuuuaccagacaaccauuaccuucgcccuauagugagucguauuag

SEQ ID NO: 125 - DNA, 18 bp, artificial Sequence
  polynucleotide sequence or in vitro generated dsRNA
atggctgttgacgtaagg

SEQ ID NO: 126 - DNA, 19 bp, artificial Sequence
  polynucleotide sequence or in vitro generated dsRNA
tgcagcttcagcttctgtg

SEQ ID NO: 127 - DNA, 20 bp, artificial Sequence
  polynucleotide sequence or in vitro generated dsRNA
accgtcgtactggtaaatcc

SEQ ID NO: 128 - DNA, 20 bp, artificial Sequence
  polynucleotide sequence or in vitro generated dsRNA
tggcggcatctccagatttg

SEQ ID NO: 129 - DNA, 19 bp, artificial Sequence
  polynucleotide sequence or in vitro generated dsRNA
ctggtcgtaccaccggtat

SEQ ID NO: 130 - DNA, 20 bp, artificial Sequence
  polynucleotide sequence or in vitro generated dsRNA
gcagagcgtaaccttcgtag

SEQ ID NO: 131 - RNA, 547 nt, artificial Sequence
  polynucleotide sequence or in vitro generated dsRNA
cuaauacgacucacuauagggagaaugcccugguucaagggauggaacguugagcgcaaggaaggcaaggcugaagguaaaugccucauugaggcccucgacgccauccugcccccugcucgccccacagacaagccccugcgucuuccccuccaggacguauacaaaaucggugguauugguacggugcccguaggcagaguugaaacugguauccucaagccugguaccaucgucgucuucgcccccgccaacaucaccacugaagucaagucuguggagaugcaccacgaagcucuccaagaggccguacccggugacaacguugguuucaacguaaagaacguuuccgucaaggaguugcgucgugguuacgucgcuggugacuccaagaacaacccacccaagggcgccgccgauuucacagcacaggucaucgugcucaaccacccuggucaaaucucaaacggauacacaccugugcuggauugccacacagcccacauugccugcaaguucgcugucucccuauagugagucguauuag

SEQ ID NO: 132 - RNA, 509 nt, artificial Sequence
  polynucleotide sequence or in vitro generated dsRNA
cuaauacgacucacuauagggagaggcccaggaaauggguaaggguuccuucaaauacgccuggguauuggacaaacugaaggcugagcgugaacgugguaucaccauugauauugcucuguggaaguucgaaaccgcuaaauacuaugucaccauuauugacgcucccggacacagagauuucaucaagaacaugaucacuggaaccucccaggccgauugcgccguacucauugucgccgcugguaccggugaauucgaggcugguaucucgaagaacggacagacccgugagcacgcucugcucgcuuucacacucggugucaagcagcugauugugggcgucaacaaaauggacuccacugagcccccauacagcgaaucccguuucgaggaaaucaagaaggaaguguccuccuacaucaagaagaucgguuacaacccagcugcugucgcuuucguacccauuucuggcuggcacggagucucccuauagugagucguauuag

SEQ ID NO: 133 - RNA, 502 nt, artificial Sequence
  polynucleotide sequence or in vitro generated dsRNA
cuaauacgacucacuauagggagaauggcuccggcaugugcaaggccgguuucgccggcgacgacgcgccccgcgccgucuucccauccaucguaggucgcccucgucaccagggugugaugguugguaugggucagaaggacuccuacguaggcgaugaggcccagagcaagagagguauccucacccugaaguaccccaucgagcacgguaucaucaccaacugggacgacauggagaagaucuggcaccacaccuucuacaacgagcugcgcgucgccccugaggaacacccaguccuccugacugaggcuccccucaacccuaaggccaacagggagaagaugacccagaucauguuugagaccuucaacucccccgccauguacgucgccauccaggcugugcucucucuguacgccucuggucguaccaccgguaucguccuggacuccggugauggugucucccacaccguucucccuauagugagucguauuag

SEQ ID NO: 134 - RNA, 592 nt, artificial Sequence
  polynucleotide sequence or in vitro generated dsRNA
cuaauacgacucacuauagggagugucaacaugggucagauaaccagagcuaccugcccaaugaaccuugcccuugcggucgucgccgagcucgacgaccucacuguuggugggcugaucaacgguuacggcaucgaggggagcucucaccucuauggccuuuucuccgacacgguugucgcgauggagguuguucucgcagauggccgggucgucagagccaccaaggacaacgaguacucugaccuuuucuauggaauucccuggucccagggaacacugggguuccuugucucugcagagaucaagcugauccccaucaaggaguacaugaagcucaccuacacuccagucaaggggggucuaaaggagaucgcgcaggccuacgcggauucuuucgcuccgagggacggugacccggcaaaggucccugacuuuguugaagggaugguguacacagagagcgagggugucaugaugacgggcguguacgcuucgaaagaagaggcgaagaagaagggcaacaagaucaacugcgugggguggugguuuaagcccugguucuaccucucccuauagugagucguauuag

SEQ ID NO: 135 - RNA, 598 nt, artificial Sequence
  polynucleotide sequence or in vitro generated dsRNA
cuaauacgacucacuauagggagagcgaguuuguggaguacaucccgacgagggaguacuaccaccggcacacccggugccuguacugggaggggaagcugauccugcccuucggcgaccaguucugguucagguuccugcugggcuggcugaugccaccgaaggugucccugcugaaggcgacccagggcgaggcuaucaggaacuacuaccacgacaaccaugugauccaggacaugcuggugccgcuguacaagguuggggaugcgcuggaguucgugcaccgcgagauggagguguauccucuguggcugugcccucaccggcuguacaagcugccggugaagacgaugguguacccggagccuggguucgagcaccagcacaggcagggcgacgcgagcuacgcacagauguucacggacgugggcguguacuacgcccccggggcggugcugaggggggaggaguucaacggcgcggaggcugugcacaggcuggagcaguggcugaucgagaaccacagcuaccagccgcaguacgcggugucggagcugaacgagaaggacuccugucucccuauagugagucguauuag

SEQ ID NO: 136 - DNA, 18 bp, artificial Sequence
  polynucleotide sequence or in vitro generated dsRNA
atggctgttgacgtaagg

SEQ ID NO: 137 - DNA, 19 bp, artificial Sequence
  polynucleotide sequence or in vitro generated dsRNA
tgcagcttcagcttctgtg

SEQ ID NO: 138 - DNA, 20 bp, artificial Sequence
  polynucleotide sequence or in vitro generated dsRNA
accgtcgtactggtaaatcc

SEQ ID NO: 139 - DNA, 20 bp, artificial Sequence
  polynucleotide sequence or in vitro generated dsRNA
tggcggcatctccagatttg

SEQ ID NO: 140 - DNA, 20 bp, artificial Sequence
  polynucleotide sequence or in vitro generated dsRNA
gtcgtggtttcccaggttac

SEQ ID NO: 141 - DNA, 20 bp, artificial Sequence
  polynucleotide sequence or in vitro generated dsRNA
gatccattcctgccctctac

SEQ ID NO: 142 - DNA, 19 bp, artificial Sequence
  polynucleotide sequence or in vitro generated dsRNA
ctggtcgtaccaccggtat

SEQ ID NO: 143 - DNA, 20 bp, artificial Sequence
  polynucleotide sequence or in vitro generated dsRNA
gcagagcgtaaccttcgtag

SEQ ID NO: 144 - DNA, 228 bp, artificial Sequence
  polynucleotide sequence or in vitro generated dsRNA
ggctgatagcacttaaggagcttcctaatcacgaaagaattctgcaggatttagttatggacatactgagagtactctctgctcctgacttagaagtccgcaagaagactttaagtctagcccttgaattagtctcttcacggaacatagaagaaatggtattagtattaacaaaggaagtgagtaaaacggtagacagtgaacatgaggatacaggaaagtacaggc

SEQ ID NO: 145 - DNA, 279 bp, artificial Sequence
  polynucleotide sequence or in vitro generated dsRNA
tacctgtggctctcacaggcagcgaagatggtaccgttagagtttggcatacgaatacacacagattagagaattgtttgaattatgggttcgagagagtgtggaccatttgttgcttgaagggttcgaataatgtttctctggggtatgacgagggcagtatattagtgaaagttggaagagaagaaccggcagttagtatggatgccagtggcggtaaaataatttgggcaaggcactcggattacaacaagctaatttgaaggcgctgccagaagg

SEQ ID NO: 146 - RNA, 501 nt, Diabrotica virgifera
gggacaaugucacaauuaaugauaauuccacaauuuccuuuuacaacagaaggacguggaaguuuguaccagaaagauccgugggagaucuuacugaucaaaucacgacuuucaauccuauuguggcaucgauagccagcuuaguuaaggacaaaaacuacauaguacuuauaggaguagacuuuuucuuggaagaauacaagaucaauuugacuguuaccaagacuguagaagaauucacuuuugaggguuacgacgauccuuugcuuaagcuaguccaaaaauuaaauauaaccgguuugaagauacccuuuaaaaaauuugggugguuuguagacagaaacgacucagcuccauacgauggaauguggaacauggacaauggagcuaauucaauugauacucuaggccuaguuagaaauuggaauuaugaaucucgugugccuuauuaugaagggacguguggagaaguggaagguacucaaggggaacuaugguauc

SEQ ID NO: 147 - RNA, 502 nt, Diabrotica virgifera
gccaacuaaaagauaauaaaacggcuugccuggaugauauacgaacagaacaaauaaagaacuuuggaccgaaaccguuaaguggcuccuaaaaaugaugaauugcuguauccguacauuacauauccccaaaaccuggaggaaagcuaaagugguagcacuauuaaaaccagggaaguguccggcagauacaaagaguuuuagaccugucucucuucugugugaccuuuucaaagugugacacugaacuugaccgccgaaucuauggagacuaaaauuauuccagaacaagcaagaaugaauaaaucauuaaacccuuaaucucauccaacauauugauuuugguuuuuaacggaaaaaauaacagguguaacguuaguagaccuaacugucgccuaugacacaguuaaccaucaacggcugcagcaaaacucuacgaaucuacaaagaauuuccgacuuacaagguuaguggaaugucgccuacagaauggacguaaagc

SEQ ID NO: 148 - RNA, 500 nt, Diabrotica virgifera
ggcauuaaaugauaaagaagaaugggugcaauuuaagguuaaaaauaacaaaaguuacagaagcuauguugaagaacaaacacgauucagaauuuuucaagaaaaucugagaaaaaucgaaaaucacaaugaaaaauauaacaauggagagucuacuuuuaaguuugguguuaccaaauuugcagaccuaacugaaaaagaauuucuggaccuguuggugcuaucuaaaaaugcaaggccuaauagaacucaugcuacacauuugcuagccccacuaagagaucuaccaucagcauuagauuggagagacaagggagcuguaacugagguaaaagaucaaggaauguguggcucuuguuggaccuuuaguacaacugggucaguagaaggagcucauuuucuuaaaacuggaaaucugguauccuuaagugaacaaaaucuaguagauugcgcaaaagacacuugcuauggguguggagguggcuggauggacaaagcuc

SEQ ID NO: 149 - RNA, 501 nt, Diabrotica virgifera
gacacgacgacacagaauucucuaaccaaaguauccuuaacgucauggagaaauucguaaagaccgucaacaaaauggaugaaaccauuuuagugccuugucguuugauggaccugaaagucggagaugagcaagacccagcuugucaaaauucaaaaaccaaaucaucccacucuguacaccaaauucuaaguucuacagaccuguuugagaucuacaauauguugaaugggguaaaggacucgcuguuauggggaggagcucaagagccuccaaagaauccuccaccaccuacuaccgcaauuguaacaucaguaacuacuccaaucgucaagggccacauccggcgacccucuucagugagugugacuuccacaaauucgucaucuacucucagcgauacugauucugagucuggcagcaaugaaaucgauucuggaaucgaugaaacgucccaagaggaaggaaaagccgaaagaaucgcucaagauuuuaaaagac

SEQ ID NO: 150 - RNA, 502 nt, Diabrotica virgifera
gaccugagugaaagccaaagagaggacaaaccagagggacccacuuugcaaguuaugccuagugagcaagucagaaaucaacuuauuaacaugucuacuguauugaaucaagccauacaagucauuaauccuaauaagaagaagcuugaacgcgaaaaacuuagagcuguuaugguucagaauuaucacgaaacaaagguuagagaacaccagaaaauuuuacaaaggcacaagauuauugaggacagaaaggaauauauugagcguuugaauacagucagggaagaagaggagcagaaaagauuggaagaaaugcaacggcagcacuuacuggccgaacaaaaacgauuggaccaagaaagagaagaaagagagcggaaacgugcucuaaaugaaauccagcagguuaaagacagacacuuaaaggaaaaacuacaacaaaucagacagacuggucauggucagaagauucugaagaaaauggaugaagacgauaucaaac

SEQ ID NO: 151 - RNA, 501 nt, Diabrotica virgifera
ggagcacccaauaauauaaauucuucuggaagaagacaucagcuguauguuggaaaucugacuugguggacaacugaucaagauauagaaaaugcagugcaugauauagggguaaccgacuuccaugaaguuaaguuuuuugaacacagagcaaauggucaauccaagggauucugugucauaucuuugggaucugagggaagcaugagacucugccuggaacuccuaucuaaaaaagagaucaauggccaaaauccccuuguuacccuucccacaaaacaagcucuuaguaacuuugaaagucagucuaaaacacgcccuucuccuacuaauaauucuaacucacguccuccccauccuaauaauaauguucauucagguccuaugcagaauuauggagguagaaugccuaugaacccuuccaugcgucccaugcccccagguaugcaaggugcuccaagaaugcaggguccaccuggauuuaauggaccaccaaacauc

SEQ ID NO: 152 - RNA, 502 nt, Diabrotica virgifera
ggguggcccaccuccagaccaccgcgcugagauuccucaguuaacagagcaagaguuugaggauauaaugucccggaauagaacaguuuccaguucggcgauugggcgggccguauccgacgccgcagcuggagaauuugcaagcgccauugagacuuugguuacugcuauuucacucaucaaacaauccaaaguggcuaacgacgaucguugcaagauccuuauaaguucgcugcaagauacuuugcguggugucgaagacaaaagcuacagcuccagccgcagagaccggucaagauccagggacagaucacauagaagaacuagaagagaacgauccucgucacgguacagagacagaagcagagagagggagcgugaacgcgauagagaucgugaucgugaacgugacagauauuaugauagauacagcgaaagagaaagagaccgagaucguucaagaagcagagaaagaacagaaagggauagagaacgagauuac

SEQ ID NO: 153 - RNA, 504 nt, Diabrotica virgifera
ggaauggaccuagaccuaaugguccugggcccaauaugggaaugagacccauggggccaccucauggacaacaagggcccccaagaccaccaaugcagggaccaccgcagcaagguccuccaagaggaaugccgccacaagguccaccgcagaugcguccagaauggaaucgaccaccaaugcaacaaggguacccucaaggcccgccgcauaugcaaggaccuaacauggguccaagagguccaccccaaaugggaccacccggggcgccucaacagcaaggaccagcuccgcacguaaauccagcauucuuucaacaaggaggaggaccaccgcccccaaugcaacacaugccuggaccagggcccgucaugccuccucaaggacccccgcaagguccaccacacggaccuguuggaccuccacacggcccaccauuggguccagcgaauguuccgccucauggaccaccucacggauaugguccaccugcagcgaugccac

SEQ ID NO: 154 - RNA, 501 nt, Diabrotica virgifera
guaauggaguuagagucaaaauugaacgaagccgaaaaagaauacauagagggcgcucccacgcgaaacaaacguaccccuucggaauggauaccgcggccgccugaaaaguucugucucacaggucaucgagcgccugugacucgaguaaucuuucauccagucuucagucucaugguuucggcaagugaagacgccaccaucaaagugugggacuucgagacuggugaauucgaacgcacccuuaaaggucacacggauugcguccaggauauagcuuuugaugcaucggguaaauuacugguauccuguagugccgacaugagcaucaaacuaugggauuuccaacagacguuugagugcgugcgcacuauguuaggucacgaucacaacguuucgagcguuucguucaugccagcuggcgauuucgucauuucgucuaguagggauaagaccaucaaaaugugggagguaucgacgggguauugcgugaaaacauac

SEQ ID NO: 155 - RNA, 502 nt, Diabrotica virgifera
gcggaauugaugauagcuuaaggcaaauugauguagaaggaaacacguacaaagcucaaagucugaaacucgguucucaaccgagagguauggauauacuuaaauccgaaaacguuauuauaacugccaguguaaaugaaauuacgguagccaaagauacccaaaaacuuagcacuuuaaaagugaauuacgaaccuuccagcguuaguuguuccucgaauggucacauugcuauuggaggaacuguagauaauaaaguacacguguucaaacucgaaaauaauaauuuggaaccaguuacagaguugacccaucucgguccuguaauggacguugccuauucaccggacgacaaguauuuaguagcuugugauggucauaggaagguaguacuguaugagacagaagaauauaagcuugccaauaaccaggaguggggauuccacaaugccagagugaacuguguugccuggucaccagacucacuauugguggcuagugc

SEQ ID NO: 156 - RNA, 501 nt, Diabrotica virgifera
gguacgaauggaaaauaaaaguguaguucuuucuucguuuuucuggggcuacauuuguuugcaaauauuugcuggacaacuuggucaaacuuaugguacuaaaugguuggcuuucguuucaauggccgucaauucaacagcuuguuucauuaucccauucauggcugaauggcugggaucuucuggaguuauagcaugucgugugguacaaggauuaucacaggguuucuuuuucccuucggugcauaauauuuugggaaaaugggccccauuggaagagagagcguuucuuucgaugauagcuuuugcaggaccaucauucgguacaauugugucacuaauugcuagcggagcaauagcaucuucuugggcaggguggccguaugcauucuacauauuuggagggcuggguuauguuuggaugcuaccgugggcauuccuugcagcgaauaccccugccuuacauccgaauauauccaaagcagaaaaagauuauauagc

SEQ ID NO: 157 - RNA, 502 nt, Diabrotica virgifera
guuaaaagugcauccacuucccuaaacucaaaaguuguuucccaacacucaagcuuuuuggguccacuugcugucgaugcaguucuuaaaauuguugaaccugguagagaacaagcuuguaauuuaucugauaucaaaguuauuaagcaacuuggagguacaguagaagauaccgaauuaguagaaggaauuuguuucccucaaagaucugcaaaugucucuggaccaaaaaggauugagaaagcuaaaauugguuucauccaguucuguauuucaccuccaaaaacagauauggaccacaaugucauuguuucugauuacgcugcuauggauagaguauuaaaagaagagagagcauauauuuugaauauugucaagcagauaaagaaagcuggauguaauguacuuuugguucaaaaaucaauuuugagggaugcaguuucagaucuugccuuacacuuuuuggauaaaaucaaguguaugguuauuaaggauauugaac

SEQ ID NO: 158 - RNA, 502 nt, Diabrotica virgifera
gcgauaaaaaugauaacaaaacggacaaguuuauuaauuuaagagacggaaaagagagcuugaaaaggaaaaagacuuuaucaguguauucgcuuccuaauuacgaugaauugaaguugacuguuuccgaauuuaaagaugauaauaaagggccauccucucuaaagacggacaaaaaaggucauccuucagaaauaucucuaccaguagaccacaaaaagacugcaacaggcucuacgggaaaguuggauacguacauaacaagaugccgaaguuuuggauccauuuucccacagcaacugaagaaauuacguccgcgaaaagcaccaacagauauugaaagcgaugauuccuuuggugguuuagaagacugggacuuaggacuaauugaacauuauaauccaaaagaugcuaguuuaccaagaccaaggaaaccaguuguuaaugaugauuccguauuagcaggccuagaaggcaugaucguaacagaagaagaaauagc

SEQ ID NO: 159 - RNA, 502 nt, Diabrotica virgifera
ggauuuucuaugucuguugucauagcuuaucuuauaaauaucuauggcagaaagacauuauguacuaugucgaguauugguauggcccuuaccaugucaguaguugcgauauacguaaaauauuaugaaauauacccagacaaagaaaaguuguuagcuacuugccacuaauuggugucauguugaacguggcauucaguaugguuggcaugcuucccguuccaugggucaugguaggagaaauguuccccuugaaagucagacccauaaugucugggauaguaguaagcuuggcgcaacuauugauauuuauuugugcaaagauuuauauaaauaugaacgacgcuuuaaacuuuagcggaacuuuaauaguauuuguaguagcuucaauuuuagcugccguuuacucaaagacgauacuaacagaaacuaaaaacaagacgcuggaagaaaucgaagcucauuuuaggggaaacaaaaaaguauguacaguugaugauac

SEQ ID NO: 160 - RNA, 501 nt, Diabrotica virgifera
gcagcuauguggaugaaacuccagauaaggagacuaaagugaaacuuauagacacauuaaggcaaguuacagaagguaaaauuuacguagaaguugaaagggcucgucugacucacaaauuagcuaaaauccgugaagaugauggugacauacaacaagcugcugacauuauucaagaacugcagguggaaacauauggaucuauggagaaaagagagaaaguggaauuaauacuagagcagaugagguuguguguugccaagcaggacuacauuagaacucagaucauuuccaagaagaucaauacuaaauucuucgaugaagauggcucuucagauuuaaaauuaaaguauuacagacugaugauggagguggaugaacaugagggcucauauuuggcaacuuguaaacauuauagggcuguucuuaauaccccaagcauuauggcagacgccgaagaaagacaagcugcagcgcaagccguuguucuuuacauuauac

SEQ ID NO: 161 - RNA, 501 nt, Diabrotica virgifera
ggaauauaauuaugaaauacgauuaaaguuuuggaaguuugaugaaucuaaacaacaauuucaccuaaauaccuccaucgaauauccgcaugaagauagcauuaauaguaugcuguuucaaccguguaguaaagaugaaagacuucagugcguaaccguuggagacgacaaaaaauuuaaaauauggcaauuguccgaaauugaaguagucacagguacucaacuauccuggcagugcuuuggaguuggcuuuuaucgaaauuugccuugcaaugcuuuaucauuuucaauagaugggucucuauuugcaacaggauucggagaaauacugacaguuuggacuucugauacauguuugcuuaaauguucucuacuccauccucuucauaagaaacaauuaaaguacauacaguuuggcuacgguaaccaaugccaucuacuuguagcggcuaguaaaaaucaacuuagcguuuggaauauccuaacguuaucuaugacauc

SEQ ID NO: 162 - RNA, 501 nt, Diabrotica virgifera
ggaagucguugaaauuaaaaaacgacgucacaggaggucggugcaacagauagauccgauggaggaaaaaagaaaaaagcuuuuagaaucacaucccuuacaaguucaaauaguggcaaaguuaaaggaugguccuuugcugacuaucaaguuuuccuaccuaauaaaauuaaaaaucauuacagucauguccagcacgaacugcucagcauguaaaauaacuggcaacucagcuagggaaguguuaaccggagagaaccuucugagugaguugguagaagaugauaauggccuagaaaguccaaauccaauaacgaaauuucagauuaagaagaucggacuuacuucuuuucaaucguuagugccacagaucggauacgcauaccauugggcucaaagaguaugcggaagagauuuucuuaauaaaaaaauggauucggaugaauuaggcagaacuaauguagaaauuauaaugaaaauaauauuuaaaagauuggaauc

SEQ ID NO: 163 - RNA, 502 nt, Diabrotica virgifera
gaucaauggacgaugaaggaaauaugaaaaaagaaucaaaugcuagaauaguaagauggucugaugggucuuacagucuacauuuaggcucugaaaucuuugacguauauaaacaaccauuacagggagaccacaaccacuuguuuauucgucaagguacagguuuacaaggucaagcaguauuccgaacaaaguugagcuuuaggccgcacucaacugaaaguuucacucacagaaagaugacucuuucuuuggcugacagaucuaccaaaacaagugguauuaaaaucaugucgcaaguugguguggauccugauuuagacaaagcaacaagaauaaagaaagaagaagaaaaacuuaggcaaucggcauccaaaccaaaaacuacuagaaagaaguccgacaaagccucuagggcacuugaaaauacuuuuguuagggaggaagaagguagugaugacgacggagcaauuucucuugcugcaauuaaaaguaaauauac

SEQ ID NO: 164 - RNA, 502 nt, Diabrotica virgifera
gcgaucaacuuauaaaacuaaacaaccaaacugcaggcagagauaaaauugccaggcugcugcaguacuugaguagguuuguauggcacaauuugcagaaaacucaaaaacaugguguaguaagucugaaaaauuuggaauuucaguugaguacuuucaggaaauuacucagauuuggaagauuugccgaaaguauauauacaacauuaccauucuucgagcaggaugaagccacuauacgcuauacugugauuuuaagcaaaauugccaauucguuguuucuuuuggcugaccacauacuaugguuaggacgugcagacguguguacaguggacacggagagauggucacgucuauccaacaaguauugguuauauuccauaacuaugaauuuaguuagagauuucuaugaaauuucuaauauuuuaaaaaguaauaaggacucaauuuuacaaaauaaauucaguucaaaggaaaugcuacauauuuuguuacgaagcuc

SEQ ID NO: 165 - RNA, 374 nt, Diabrotica virgifera
gaugggcgaggaggaaaucacaccaaauaauaucaaagaaaaucagagugagaauaugaaugggaauauaaauggucaagaggaaaauccaccuccagaagaaauggauacaaauggggaaaaugauguaaaugaagaugaucuggaugaagacaaugaugacaugucgccugaagaguuugcugcacuugaucaccaguuagaugccuuaaauucugcuuuagaugacauagaacagaaaaaugauaauauacauucgcaguuacuagaacuacuccaugcuaacagggaaauccggacucaauuacagcaagauaaagcuagcacagauaacagagaagacguaaauaaaacaaaugaaccaaaagcaugac

SEQ ID NO: 166 - RNA, 500 nt, Diabrotica virgifera
gcagguuauuaguacauuaacgaaaguucuuaaauguaaucagagaagcucaacagaguuuguuacgaacaucgaccgggaagguagagccaucgugaaauguucaucuuuucagcacugcugcgaucuuaaacaagauaucgagaaguuuacgucccgacacggcaacaaaccuuugaagguacuuguuaaccaugcucaucuuauaucucaucagauauuugcaggaaagauauuaaauuggcuagaaaaggucuuaauacaaggagaaggauucagagcuauuuuugccgauguugugcugaagccacagaauccagagccgugcauaauaaagggcauccuacaaaaagauuuaggccuuuggaagagcgcuaggagccaauggcaucgcuuguuaauaucaggcaugaugcucgaguaugagaacaagaaagcuuuagcuaaaauauuuaccaaaaacuaugggcaaguaaugaaagacuuuaucaaagaugauc

SEQ ID NO: 167 - RNA, 502 nt, Diabrotica virgifera
gugaaauauuacuugcuaguguucuguauagcaacuacacuuacauuaucuacggcacaauccuaugaagacaagagauguaaguguauaugccccaguauauccucaguaguaacgaauaagacggaaucuaagaaccacacaucuaggauuuuauacauuaccaauguaccaccaaauaaaugcaauugugaugaaguuauacuaccuaggauuagucaagauauuauaggaaaagaacaagaauuuuguccaagaugugaaugcaaauaugaaaauagaaacacuacuauaauuaaaguaguggugauuauaguaauuuggguuauuucgauuuuggucauauacauggcauucuugaucauacuggacccgcugcugaacaagaggauuaaaggaaacuaccaagagcauacaaaugaagaggaugacguaucugcugguccaaugucccacaacaugagcguaagaggaaacgucuugaacagaguuggacaucaac

SEQ ID NO: 168 - RNA, 501 nt, Diabrotica virgifera
ggcuguuaauucaauuuuaaggcauguugcggaauuacuaaaguaugaaucagaugaacaauuagaagaauuguaucagaagacugcuugguauuucgaagaaaaguauaagaagaauaaagcuagugcauaugacuucuucaaacaggcuguuuuagaccccaguauuuuagcagaaugugaauuagaugacaaaacaaaagaagucuugcuuaguaacauuaagagaaagcuaacaucucaagcagucaaaaucagagcugauauugaaugugcuuguuaugguuaugaagguaucgaugcuguuaaaacugcucuuaaagcuggcuuggcucuuucaacagaagaauuacccauuaaaauaaaucuuauagcuccuccucucuauguuaugacuacaucuacaccugaaaaacaagaugguuuaaaaguuuuaggagaugcuauagaaaaagucaaagcgacaaucacggaauuggguggaguauuuaauauucaaac

SEQ ID NO: 169 - RNA, 500 nt, Diabrotica virgifera
guauaagaagaauaaagcuagugcauaugacuucuucaaacaggcuguuuuagaccccaguauuuuagcagaaugugaauuagaugacaaaacaaaagaagucuugcuuaguaacauuaagagaaagcuaacaucucaagcagucaaaaucagagcugauauugaaugugcuuguuaugguuaugaagguaucgaugcuguuaaaacugcucuuaaagcuggcuuggcucuuucaacagaagaauuacccauuaaaauaaaucuuauagcuccuccucucuauguuaugacuacaucuacaccugaaaaacaagaugguuuaaaaguuuuaggagaugcuauagaaaaagucaaagcgacaaucacggaauuggguggaguauuuaauauucaaauggcucccaaaguggucacagcuaccgacgaagccgaacucgucaaacagauggaacgagcugaacucgaaaacgcagaaguugcuggcgacgacgacgaagaac

SEQ ID NO: 170 - RNA, 502 nt, Diabrotica virgifera
gcguaauaucuaacaauuuaggaaguguguccuccacaucuauagaucccaauucagguuuagcuaguaugguuccuggaguacaaacaccggguaugcuaacacccacaggcgacauggaucugcgcaaaaucggccaagcaagaaacacucugaugaauguuaaacugucacaaguaucugacucuguaaccggucaaacaguuguugauccuaagggguaucuuacugauuuacaaucuaugauacccacuuauggaggugacauuaaugacaucaagaaagcuagacuacuauuaaaaucagucagagaaacuaauccaaaucauccaccugcuuggauugccagugcuaggcuagaggagguuacaggcaaaguccaagcagcuagaaaccuuauaaugaaaggcugugaaguaaauccccaaagcgaggaccuauggcuugaagcggcuagacuaaauccaccugauaccgcuaaagcaaucauugcucaagcagc

SEQ ID NO: 171 - RNA, 496 nt, Diabrotica virgifera
gacagcaaaaauuaauuuucagguaaaaaauaaagauauucugcaaagugguauauuuaaucaaacuuuaagggacuggcagaguauccaaugugaaaucacagcgaaaaauuugauguacccagucuuuauuguggaagaugaugaugucguacaacccauuaguaguaugccuggaauuucaagguauggaguaaauaaauuacgugaucauuuacaagauguuguuaaaaauggacuacaaucuguguuacuuuuuggagugguagaaaaguuguccaaggaugauuuugcuacccacgcagauagcucacaaaauccaguagucagggcacuuccuaaacuaaaaaaaugguuuccuaaucugacaauagccugugauguuuguuuaugcccuuacaguucccauggacauuguggaauacugaacaaugaugguaguuuaaauaauacugcuaguauccaaagaauaucagauguagcucuagcuuaugcc

SEQ ID NO: 172 - RNA, 502 nt, Diabrotica virgifera
gggguguuauuuaucgaaaaacccgaucugguaaucuggagaagacuucaccauucuggaucaggucaauacgaauauaaaguguaugguacuuacaaugaugugucagccgaagauuuuuugaauguucaaguugauauugacuauaggaggaagugggauacgagugcaguuauccuugaacacgcagagucugauccuuugaagaauucuaacagcgaugucauuuacugggaacuuuuauggccuaggcuguuugugaaucgagauuacgucuuuaacagacguuacuugauagacaacacauugaacacuauauucauccuaaaccggagcaccgaacauccaaaguuuccaaaauacgcagaaaaauaucggauagacgacuauuggucguguaugguaaucaaaccguaugaaggagacaugacgaggccaggaauacaguucgucuugaccuacuacgacaacccaggcgugaguauaccauccucgguaacac

SEQ ID NO: 173 - RNA, 496 nt, Diabrotica virgifera
gugguacagcaaucaaauguaaacgauuauuuacuaaaaaaacaacaagaaaguccuaaagaauuaggcucagaaugggccgaacuugaagaacuucauaauaaaaaauuguggcaucaguugacucuaaaauugcugaauuuuauuaagaaaccagaacuacagaagaaugauaaccucauacaacuguacaauaacuuuauucaaaguuuugaaaauaaaaucaauccuuugucauugguugaaauuguugcuauaguaguccaacaauucaaaaauccaaaagaugcugucgcuuuucuugaaaagacugaaccuaagguuaaaauuaauucagaugcccaaaacuugugcaaaguuuuagcugggcagauauauaucgaaaaguugaacgauuuagaugcuacuaaaaagauaauugaagaaguggaaucuacauuggacaaugcugaugguguuacuccaguucauggaagauuuuauuuacuugccucac

SEQ ID NO: 174 - RNA, 502 nt, Diabrotica virgifera
guaguagcaaucuuaaacacaggcuuguucaaaaucuacccagaucaacaucauuuuggaguacaauugauagaugaaggugcagauauauucgaugccaaaaucaaccucgaaguccagugguguacggaacauauuauagcagcaaucgagagaaaaggugguguuaucacuuccgcuuacuacgauccucacagucugcaggcuaugguuaacagcaagaaguuuuuugaaagagguauuccaauaccccgcagaaugaugccucccccagacgccauagaacacuacucagauccugcacagaggggauauuuggcagaucccgagaagauaucccaagagcgucuaguccuagcccagaaauaugguuacagguuaccaaaaauagaagaagauccugcauacgagauguuaauggaaaggaaagauccuaggcagauauucuauggucuacaucccggauggguggucaauuugacggauaagacuauacuuaaac

SEQ ID NO: 175 - RNA, 502 nt, Diabrotica virgifera
gaaguggguaaacuaaaaauuagcaaaccuguuggacaaaaggcucaaguuucgcuuacauuaucuucagcaauucuuaauuugaaugagccuggacaagaaaguauuccaaaggaucauagauuagauguauccacaguuacucaacaaacuuugggugucuuuucacauguuacaccaacuaauauugauucugugguaccugaaacugaaaagcugcacauggaaggcaaaauagugcaaaaauuggaaugcaggccauaugcagauaauuguuacaugaaguugaaauuagaaucuauuaggaaagcuucucuaccaguucgccaagugaagcaguuagacaggguuguacaaacauacaagccaguaucugaucauaaaaauaauauugaguacauggagagaaagaaagcugaagguaaaaaggcucgugaugacaaagaagcuguuuuggacauguuguuugcagcuuucgaaaagcaccaauauuauaacauac

SEQ ID NO: 176 - RNA, 501 nt, Diabrotica virgifera
guaacaaucaaagcucaagaugaugccgacauaguaacguuuauguuugaagccaaaaagcaggacaagaucucagauuacgaaaugaaacugaugaauuuggaccaggagcauuuggguaucccagaaacagauuucucuugugucaucaggaugccugcagcugaauucgcaagaauagucaaagaucuuucacaguuuggagaaucuaucguaaucucaugcacaaaagaggguguuagguucucaacuucuggagauauuggcagugcuaacaucaaaauugcccagacaaguaauuucgaaaaggaagaggaaucuguaagcauagaaaugcaagaaccaguuacucuuacuuucgcuugucaguauuugaauuccuucaccaaagccacaccucuuacuaacguugugcagcuaucgaugucugacaauguaccuuuaguaguugaauaucaaauaccugauuugggccauuugagguacuacuuagcaccuaac

SEQ ID NO: 177 - RNA, 502 nt, Diabrotica virgifera
gaguaaugaugacacaguaacaaucaaagcucaagaugaugccgacauaguaacguuuauguuugaagccaaaaagcaggacaagaucucagauuacgaaaugaaacugaugaauuuggaccaggagcauuuggguaucccagaaacagauuucucuugugucaucaggaugccugcagcugaauucgcaagaauagucaaagaucuuucacaguuuggagaaucuaucguaaucucaugcacaaaagaggguguuagguucucaacuucuggagauauuggcagugcuaacaucaaaauugcccagacaaguaauuucgaaaaggaagaggaaucuguaagcauagaaaugcaagaaccaguuacucuuacuuucgcuugucaguauuugaauuccuucaccaaagccacaccucuuacuaacguugugcagcuaucgaugucugacaauguaccuuuaguaguugaauaucaaauaccugauuugggccauuugagguac

SEQ ID NO: 178 - RNA, 501 nt, Diabrotica virgifera
gaggaauccagcucgaacagcgacagcucugauaauucaguaaaauugcuggaaaagcucacaaaagaaagaauuagacuuggagaagaaaggaagaagcaaaaagaacuaaucaaagcuacugaaacagcagaggagaagagaaugaggcggcucguaaagaaggagaacaaagagagauccaggaaagagagaaugggcugggauaacgaguauuuacauuauacaaacagugacaauccuuucggggauggaaacuuguugucuacauuugugugguccaagaaguuaaacaaagaaggauugaaagguguuagucaagaagaaaucgaagcaauaaacaggaugaaacaagaagaaaacaaaagagaacuggaaaaaguaaaaaagagacgucuagaaagagaauuagaaagacagaagagggacgaagaaacccagaugcuccaaagaagcaaggaagcagcacaauuugaagagugggagaggcaagaagauaac

SEQ ID NO: 179 - RNA, 501 nt, Diabrotica virgifera
gaacagucuggaagaaauauuuuggacuaccagaaucaggcgaaaauguuauuucgaaaauuggggcaccaguccccugcuagauguucaauugaaacgggaccuuauauauuccauuauuuaauagaauacgaaguuuguuaccuaguauuaugugaaaaggcuuucucaaaacgacuggcuuacucauauuuggaagauauagcacaagaauuccacgcacaauauggcaaaagagugaauacaguaacuaggccuuauacauucauagaguuugacacauauauccagaaagccaaaaaacaguuugcagauucgagaucgagaaggaauuuaaaugugauaaauaaucagcuacacgauguccaaaggauuaugguacaaaauauagaugaugugcugcagcgaggaacuguucuaucagaguuggacaccaaaacgcagaaucuauccauguuaacggacaaauacaagaaggauucgacauacuugaacacaaac

SEQ ID NO: 180 - RNA, 482 nt, Diabrotica virgifera
gauggaugcugaaacuggagaauuuuaccuagaccuugaaacuggagaaauauccgaagcccccgcaguccaaaaugucgaaacgggggaguacgaauauaccagaacuuuuaaaaucccaagcuacuacuacagaagauaccaagaaagaaaagaaaaaaccaacugcacuccacguaaagcagauccccuggagucacaguugauuaccgcggcuaucuuucuacuaccgacaaugauauucuuccaucccaucaugcucguuuuuguuugcgugauagaaauauuuuuacauacucgcauucacagaaagaacaaagaacuagaagaucuguccuuuuauuaccagagcccauuacauggccuuacaaaagagguaugugcuagauguaaagacgaaaaagccaagaauaagaucgcgaagcugcaagacaagcagcaugagaaauucaagaauuacaucaaaaggguuguaacuuaac

SEQ ID NO: 181 - RNA, 501 nt, Diabrotica virgifera
ggugaauauaaugacucugauauugaaugggaacuguguuuuccccaagcacaaagauaucuggaaaguuucaugagucaugcucaaaugaaaagcuugaucauucuucuaacacuucauaaaacuuucauagaaccucagacugcgcauuuaggucucacggccgaucauauaagaaacuucaucuuuuuggaaugugagucccauuauagugacugggcagaacauaggcuagguauuaaauuguugaaaguacucaaacgucuucauacacaucuaucacaagcuaaaccauguauuccagacuuuuuuguuaccaauaaaaauacuuuaagugaaguaccuauuagaaaauaagaagagcucuaauggcuuuggaugaaauuuuacaaucuccccugauguacuucauaaaagccuuacgaaaucuuagauauacagacgggagaaauuucuucccuccuuuaaauuuuaaacaguugcacgaucugcuaaauaaac

SEQ ID NO: 182 - RNA, 502 nt, Diabrotica virgifera
gccaaauuauuuaaagauaacgacgcaaaauguguacuuggcuauuuacaaacuagacacaagaaagaugauuccaguuuaucgucuuuauuuguuccuguucaaauuaaaccgagugcagaugacauaaauguuggagcagaacuuacaggaacuuugaacaaaacagauuuguuaaaaguuuugaauaaguuuuaucagaaaaaagaaauuaaggcauugcuaguagauaauggauuagaucaguaccuucagcaccaagccuaugugaguuuccgaagauauugccuagaagcacaaaauuuaccagcagauauccacguagucuucagugacauucuacagggagcuggaaauaucacugauauuuuccccuacuuucuacgacaugccaaaaugauguuuccccaucucgacugcauggaugaucuuagaaaaauuucugauuuaagaucaccugcuaacugguauccugaagcaagggcuauuaacagaaaauaac

SEQ ID NO: 183 - RNA, 501 nt, Diabrotica virgifera
ggagaacauuuaacucuaaaaauuaggucgaaaacauuugaagcaauguuaagacaggaaauuggcugguaugaccaaaaaagcaauggaguuggggcacugugugcacgucuggcuggagaugcuguagcuguccaaggggcagcugggccacagauaggaacaacaauaaacuuuauuucaacauucauacuuacguguacguucucguuuuauuuugaguggaggacaagcuuugugcuuuuuucuuugugucccguaauauucuuuucuguauauuuugagcagaagguauuacaagaggaugccacgaaaaaccaaaaaauguuagaagcaucugcaaaguuggcuguagaagcuaucgguaauauaagaacagugguuucucuagguugugaaaaaguauuuauggaacaguauaucaaagaguuauuaccguaucagaaaauggcaagaaaaaagucacauuaucguggcauaauaguagguuuagcuagaagc

SEQ ID NO: 184 - RNA, 490 nt, Diabrotica virgifera
gauggauaaugaucuugacagguccauucgcuuauuggaaaaugcuuuaucuaccucuaacagaggucuuuucaagaagucauuuggaaaaucaaaguuagcuacugacaauauuucuaauguguccauagcuucugcagaugaugauuuaaggauaucaucaguaaaagcuuccuuaccagcgauaaugcagugucuaggauacugcagucugaucaaacuguaacuggaaauguucuucaagccaguacagcaccuuggaaaacggcucuggauagucuuuauaccgaauuuuuugaaauacuuacuucacacucagguggcuuugauauacuggaaguaguuaccgacuuagcuagguguugcucugaugcccuuaaaguaauucagaguuugaagucgaagguagcaguuucgcaguuagaagaagaaauaaguuuagagaaggaaaggaauacauggagauugcuuuuuauccuuuaccaagauc

SEQ ID NO: 185 - RNA, 508 nt, Tomato Golden Mosaic Virus
gcucacaaaagaugaagcguuagagcaauuacagucaauacaacuaacuucgaauaaacguuauaucaagauuugcagagagcuucacgagaauggggaaccucauauccaugcccuuauccaacuugaagggaaaguccagaucaccaacgaacgacaguucgaccugguauccccaaccaggucagcauauuuccauccgaacauucagggagcuaaaucuaguuccgacgucaaaucauacaucgacaaagauggagauacccucgaauggggagaauuccaaaucgacggcagaucugcuaggggaggccagcagacugcaaacgauucauaugcaaaggcgcuuaacgcaguuggagugcaagaagcacuccaaauuuuaaaggaagaacaaccuagggauuuuguuaaagauuuucacaaucucaaggguaaccuugagaagauauuuucaaaggcuccagaaccguggguuccuccauuuccacuuuccucauuuaauaac

SEQ ID NO: 186 - RNA, 440 nt, Tomato Golden Mosaic Virus
gccagaggaguuacagacaugggcugaugauuauuuuggaaauggugccgcugcgcggacuuuaagaccuaucaguauuaucaucgaaggugauucaagaacuggaaaaacaaugugggcucguucauuaggaauucauaauuaucugaguggucaucuagauuucaauucuaggguuuacucaaauaauguuauguacaacgucauugaugacguaccaccgcauuaucuaaagaugaaacacuggaaagagcucauuggggcccagacagacuggcagaccaacuguaaauacgggaaacccauucaaauuaaagguggcauuccaucaaucgugcuaugcaauccuggugagggggcuagcuauaaauacuaccucgacaaacaggaaaacucacaucucaaggcguggacacuucacaaugcaaaauucgucuucc

SEQ ID NO: 187 - RNA, 500 nt, Cauliflower Mosaic Virus
gaaucaaccagugcuggucguaaccgucgacgucguccgcgucgugguucccgcuccgcccccuccuccgcggaugcuaacuuuagagucuugucgcagcagcuuucgcgacuuaauaagacguuagcagcuggucguccaacuauuaaccacccaaccuuuguagggagugaacgcuguagaccuggguacacguucacaucuauuacccuaaagccaccaaaaauagaccgugggucuuauuacgguaaaagguuguuacuaccugauucagucacggaauaugauaagaagcuuguuucgcgcauucaaauucgaguuaauccuuugccgaaauuugauucuaccgugugggugacaguccguaaaguuccugccuccucggacuuauccguugccgccaucucugcuauguucgcggacggagccucaccgguacugguuuaucaguaugccgcaucuggaguccaagccaacaacaaacuguuguaugaucuuuc

SEQ ID NO: 188 - RNA, 501 nt, Cauliflower Mosaic Virus
gucguccaacuauuaaccacccaaccuuuguagggagugaacgcuguagaccuggguacacguucacaucuauuacccuaaagccaccaaaaauagaccgugggucuuauuacgguaaaagguuguuacuaccugauucagucacggaauaugauaagaagcuuguuucgcgcauucaaauucgaguuaauccuuugccgaaauuugauucuaccgugugggugacaguccguaaaguuccugccuccucggacuuauccguugccgccaucucugcuauguucgcggacggagccucaccgguacugguuuaucaguaugccgcaucuggaguccaagccaacaacaaacuguuguaugaucuuucggcgaugcgcgcugauauaggugacaugagaaaguacgccguccucguguauucaaaagacgaugcgcucgagacggacgagcuaguacuucauguugacaucgagcaccaacgcauucccacaucuggagugc

SEQ ID NO: 189 - RNA, 501 nt, Tomato Spotted Wilt Virus
gcauuguugcuuuguugacacaaggcaaagaccuugaguuugaggaagaucagaaucugguagcauucaacuucaagacuuuuugucuggaaaaccuugaccagaucaaaaagaugagcguuauuucaugucugacauuccugaagaaucgucagagcauaaugaagguuauuaagcagagugauuuuacuuuugguaaaauuaccauaaagaaaacuucagacaggauuggagccacugacaugaccuucagaaggcuugauagcuugaucagggucaggcuuguugaggaaacugggaauucugagaaucucaauacuaucaaaucuaagauugcuucccacccuuugauucaagcuuauggauuaccucuugaugaugcaaagucugugaggcuugccauaaugcugggagguagcuuaccucuuauugcuucaguugauagcuuugagaugaucaguguugucuuggcuauauaucaggaugcaaaauacaaggacc

SEQ ID NO: 190 - RNA, 501 nt, Tomato Spotted Wilt Virus
gaccuucagaaggcuugauagcuugaucagggucaggcuuguugaggaaacugggaauucugagaaucucaauacuaucaaaucuaagauugcuucccacccuuugauucaagcuuauggauuaccucuugaugaugcaaagucugugaggcuugccauaaugcugggagguagcuuaccucuuauugcuucaguugauagcuuugagaugaucaguguugucuuggcuauauaucaggaugcaaaauacaaggaccucgggaucgacccaaagaaguaugacaccagggaagcuuuaggaaaaguuugcacugugcugaaaagcaaagcauuugagaugaaugaagaucaggugaagaaggggaaagaguaugcugcuauacuuagcuccagcaauccuaaugcuaaaggaaguauugcuauggaacauuacagugaaacucuuaacaaguucuaugaaauguuugggguuaaaaaacaggcgaaacucacagaacuugc

SEQ ID NO: 191 - DNA, 20 bp, artificial Sequence
  polynucleotide sequence or in vitro generated dsRNA
cccaggtcatcatcatgaac

SEQ ID NO: 192 - DNA, 20 bp, artificial Sequence
  polynucleotide sequence or in vitro generated dsRNA
gagctcagcaaacttgacag

SEQ ID NO: 193 - DNA, 18 bp, artificial Sequence
  polynucleotide sequence or in vitro generated dsRNA
aggctttcgctgcgtgtt

SEQ ID NO: 194 - DNA, 19 bp, artificial Sequence
  polynucleotide sequence or in vitro generated dsRNA
tggcccatccaaactcaga

SEQ ID NO: 195 - DNA, 20 bp, artificial Sequence
  polynucleotide sequence or in vitro generated dsRNA
gctcaagttcttcggatgac

SEQ ID NO: 196 - DNA, 20 bp, artificial Sequence
  polynucleotide sequence or in vitro generated dsRNA
acttcttccagcagactagc

SEQ ID NO: 197 - DNA, 20 bp, artificial Sequence
  polynucleotide sequence or in vitro generated dsRNA
gcaaccactcccaaatactc

SEQ ID NO: 198 - DNA, 20 bp, artificial Sequence
  polynucleotide sequence or in vitro generated dsRNA
cagggttgtacccaactttc

SEQ ID NO: 199 - DNA, 20 bp, artificial Sequence
  polynucleotide sequence or in vitro generated dsRNA
tctggcatcacaccttctac

SEQ ID NO: 200 - DNA, 20 bp, artificial Sequence
  polynucleotide sequence or in vitro generated dsRNA
ttctcacggttagcctttgg

SEQ ID NO: 201 - DNA, 20 bp, artificial Sequence
  polynucleotide sequence or in vitro generated dsRNA
tgtcctgccatctctatctc

SEQ ID NO: 202 - DNA, 20 bp, artificial Sequence
  polynucleotide sequence or in vitro generated dsRNA
acatccgaatggtctctacg

SEQ ID NO: 203 - DNA, 20 bp, artificial Sequence
  polynucleotide sequence or in vitro generated dsRNA
cacaaccgtgcagtttacag

SEQ ID NO: 204 - DNA, 20 bp, artificial Sequence
  polynucleotide sequence or in vitro generated dsRNA
aaatgcgcccaagcatatcg

SEQ ID NO: 205 - DNA, 20 bp, artificial Sequence
  polynucleotide sequence or in vitro generated dsRNA
cagaggacgaggaatatgag

SEQ ID NO: 206 - DNA, 20 bp, artificial Sequence
  polynucleotide sequence or in vitro generated dsRNA
ctagcagcattgtcagtagg

SEQ ID NO: 207 - DNA, 20 bp, artificial Sequence
  polynucleotide sequence or in vitro generated dsRNA
cggtgttcgacagcagctac

SEQ ID NO: 208 - DNA, 20 bp, artificial Sequence
  polynucleotide sequence or in vitro generated dsRNA
cttcgccgccaacaataccc

SEQ ID NO: 209 - DNA, 22 bp, artificial Sequence
  polynucleotide sequence or in vitro generated dsRNA
gcgcaagtttttcgtagatgac

SEQ ID NO: 210 - DNA, 21 bp, artificial Sequence
  polynucleotide sequence or in vitro generated dsRNA
accatagtccacagatgacac

SEQ ID NO: 211 - DNA, 20 bp, artificial Sequence
  polynucleotide sequence or in vitro generated dsRNA
gctgcgtgttgtgcgttctg

SEQ ID NO: 212 - DNA, 20 bp, artificial Sequence
  polynucleotide sequence or in vitro generated dsRNA
tcgtcgcgtgctgtctgttc

SEQ ID NO: 213 - DNA, 18 bp, artificial Sequence
  polynucleotide sequence or in vitro generated dsRNA
aggctttcgctgcgtgtt

SEQ ID NO: 214 - DNA, 19 bp, artificial Sequence
  polynucleotide sequence or in vitro generated dsRNA
tggcccatccaaactcaga

SEQ ID NO: 215 - DNA, 20 bp, artificial Sequence
  polynucleotide sequence or in vitro generated dsRNA
gctcaagttcttcggatgac

SEQ ID NO: 216 - DNA, 20 bp, artificial Sequence
  polynucleotide sequence or in vitro generated dsRNA
acttcttccagcagactagc

SEQ ID NO: 217 - DNA, 19 bp, artificial Sequence
  polynucleotide sequence or in vitro generated dsRNA
ggatgctactcgccagaca

SEQ ID NO: 218 - DNA, 19 bp, artificial Sequence
  polynucleotide sequence or in vitro generated dsRNA
gtggtcagcctgcttcaac

SEQ ID NO: 219 - DNA, 22 bp, artificial Sequence
  polynucleotide sequence or in vitro generated dsRNA
gcgcaagtttttcgtagatgac

SEQ ID NO: 220 - DNA, 21 bp, artificial Sequence
  polynucleotide sequence or in vitro generated dsRNA
accatagtccacagatgacac